European Patent Application EP 4 257 599 A2, published October 11, 2023. Title: Rodents having an engineered heavy chain diversity region. Applicant: Regeneron Pharmaceuticals, Inc. Application EP. The sequence listing filed with the application follows.

SEQUENCE LISTING (245 sequences)

SEQ ID NO: 1 - DNA, 150 bp, Homo sapiens
  source 1..150: mol_type = genomic DNA
atggcagctactgccagcccgcagccactggctactgaggatgccgattctgagaatagcagcttctactactatgactacctggatgaagtagctttcatgctctgccggaaggatgctgtggttagctttggcaaagttttcctgcca

SEQ ID NO: 2 - protein, 50 aa, Homo sapiens
MAATASPQPLATEDADSENSSFYYYDYLDEVAFMLCRKDAVVSFGKVFLP

SEQ ID NO: 3 - DNA, 15 bp, Homo sapiens
  source 1..15: mol_type = genomic DNA
agcttcttgtgcaag

SEQ ID NO: 4 - protein, 5 aa, Homo sapiens
SFLCK

SEQ ID NO: 5 - DNA, 102 bp, Homo sapiens
  source 1..102: mol_type = genomic DNA
caaacccatgaaaaccccaagggagtttggaactgccatgccgatttcggcgggcatggcaccatttggaagctcttcctccggttccagcagaacctgcta

SEQ ID NO: 6 - protein, 34 aa, Homo sapiens
QTHENPKGVWNCHADFGGHGTIWKLFLRFQQNLL

SEQ ID NO: 7 - DNA, 66 bp, Homo sapiens
  source 1..66: mol_type = genomic DNA
ctgcataccctgctggacctgcaagtattcggcaactgtgaggttagccagcatctagactatgcc

SEQ ID NO: 8 - protein, 22 aa, Homo sapiens
LHTLLDLQVFGNCEVSQHLDYA

SEQ ID NO: 9 - DNA, 150 bp, Homo sapiens
  source 1..150: mol_type = genomic DNA
atggcagctactgccagcccgcagccactggctactgaggatgccgattctgagaatagcagcttctactactatgactacctggatgaagtagctttcatgctcagccggaaggatgctgtggttagctttggcaaagttttcctgcca

SEQ ID NO: 10 - protein, 50 aa, Homo sapiens
MAATASPQPLATEDADSENSSFYYYDYLDEVAFMLSRKDAVVSFGKVFLP

SEQ ID NO: 11 - DNA, 15 bp, Homo sapiens
  source 1..15: mol_type = genomic DNA
agcttcttgagcaag

SEQ ID NO: 12 - protein, 5 aa, Homo sapiens
SFLSK

SEQ ID NO: 13 - DNA, 102 bp, Homo sapiens
  source 1..102: mol_type = genomic DNA
caaacccatgaaaaccccaagggagtttggaacagccatgccgatttcggcgggcatggcaccatttggaagctcttcctccggttccagcagaacctgcta

SEQ ID NO: 14 - protein, 34 aa, Homo sapiens
QTHENPKGVWNSHADFGGHGTIWKLFLRFQQNLL

SEQ ID NO: 15 - DNA, 66 bp, Homo sapiens
  source 1..66: mol_type = genomic DNA
ctgcataccctgctggacctgcaagtattcggcaacagtgaggttagccagcatctagactatgcc

SEQ ID NO: 16 - protein, 22 aa, Homo sapiens
LHTLLDLQVFGNSEVSQHLDYA

SEQ ID NO: 17 - DNA, 135 bp, Homo sapiens
  source 1..135: mol_type = genomic DNA
atggcagctactgccagcccgcagccactggctactgaggatgccgattctgagaatagcagcttctactactatgactacctggatgaagtagctttcatgctctgcgaggttagccagcatctagactatgcc

SEQ ID NO: 18 - protein, 45 aa, Homo sapiens
MAATASPQPLATEDADSENSSFYYYDYLDEVAFMLCEVSQHLDYA

SEQ ID NO: 19 - DNA, 81 bp, Homo sapiens
  source 1..81: mol_type = genomic DNA
ctgcataccctgctggacctgcaagtattcggcaactgtcggaaggatgctgtggttagctttggcaaagttttcctgcca

SEQ ID NO: 20 - protein, 27 aa, Homo sapiens
LHTLLDLQVFGNCRKDAVVSFGKVFLP

SEQ ID NO: 21 - DNA, 78 bp, Homo sapiens
  source 1..78: mol_type = genomic DNA
agcttcttgtgccatgccgatttcggcgggcatggcaccatttggaagctcttcctccggttccagcagaacctgcta

SEQ ID NO: 22 - protein, 26 aa, Homo sapiens
SFLCHADFGGHGTIWKLFLRFQQNLL

SEQ ID NO: 23 - DNA, 39 bp, Homo sapiens
  source 1..39: mol_type = genomic DNA
caaacccatgaaaaccccaagggagtttggaactgcaag

SEQ ID NO: 24 - protein, 13 aa, Homo sapiens
QTHENPKGVWNCK

SEQ ID NO: 25 - DNA, 135 bp, Homo sapiens
  source 1..135: mol_type = genomic DNA
atggcagctactgccagcccgcagccactggctactgaggatgccgattctgagaatagcagcttctactactatgactacctggatgaagtagctttcatgctcagcgaggttagccagcatctagactatgcc

SEQ ID NO: 26 - protein, 45 aa, Homo sapiens
MAATASPQPLATEDADSENSSFYYYDYLDEVAFMLSEVSQHLDYA

SEQ ID NO: 27 - DNA, 81 bp, Homo sapiens
  source 1..81: mol_type = genomic DNA
ctgcataccctgctggacctgcaagtattcggcaacagtcggaaggatgctgtggttagctttggcaaagttttcctgcca

SEQ ID NO: 28 - protein, 27 aa, Homo sapiens
LHTLLDLQVFGNSRKDAVVSFGKVFLP

SEQ ID NO: 29 - DNA, 78 bp, Homo sapiens
  source 1..78: mol_type = genomic DNA
agcttcttgagccatgccgatttcggcgggcatggcaccatttggaagctcttcctccggttccagcagaacctgcta

SEQ ID NO: 30 - protein, 26 aa, Homo sapiens
SFLSHADFGGHGTIWKLFLRFQQNLL

SEQ ID NO: 31 - DNA, 39 bp, Homo sapiens
  source 1..39: mol_type = genomic DNA
caaacccatgaaaaccccaagggagtttggaacagcaag

SEQ ID NO: 32 - protein, 13 aa, Homo sapiens
QTHENPKGVWNSK

SEQ ID NO: 33 - DNA, 216 bp, Homo sapiens
  source 1..216: mol_type = genomic DNA
atggcagctactgccagcccgcagccactggctactgaggatgccgattctgagaatagcagcttctactactatgactacctggatgaagtagctttcatgctctgccggaaggatgctgtggttagctttggcaaagttttcctgccactgcataccctgctggacctgcaagtattcggcaactgtgaggttagccagcatctagactatgcc

SEQ ID NO: 34 - protein, 72 aa, Homo sapiens
MAATASPQPLATEDADSENSSFYYYDYLDEVAFMLCRKDAVVSFGKVFLPLHTLLDLQVFGNCEVSQHLDYA

SEQ ID NO: 35 - DNA, 117 bp, Homo sapiens
  source 1..117: mol_type = genomic DNA
agcttcttgtgcaagcaaacccatgaaaaccccaagggagtttggaactgccatgccgatttcggcgggcatggcaccatttggaagctcttcctccggttccagcagaacctgcta

SEQ ID NO: 36 - protein, 39 aa, Homo sapiens
SFLCKQTHENPKGVWNCHADFGGHGTIWKLFLRFQQNLL

SEQ ID NO: 37 - DNA, 105 bp, Homo sapiens
  source 1..105: mol_type = genomic DNA
atggcagctactgccagcccgcagccactggctactgaggatgccgattctgagaatagcagcttctactactatgactacctggatgaagtagctttcatgctc

SEQ ID NO: 38 - protein, 35 aa, Homo sapiens
MAATASPQPLATEDADSENSSFYYYDYLDEVAFML

SEQ ID NO: 39 - DNA, 42 bp, Homo sapiens
  source 1..42: mol_type = genomic DNA
cggaaggatgctgtggttagctttggcaaagttttcctgcca

SEQ ID NO: 40 - protein, 14 aa, Homo sapiens
RKDAVVSFGKVFLP

SEQ ID NO: 41-42 - skipped (2 entries)

SEQ ID NO: 43 - DNA, 33 bp, Homo sapiens
  source 1..33: mol_type = genomic DNA
caaacccatgaaaaccccaagggagtttggaac

SEQ ID NO: 44 - protein, 11 aa, Homo sapiens
QTHENPKGVWN

SEQ ID NO: 45 - DNA, 66 bp, Homo sapiens
  source 1..66: mol_type = genomic DNA
catgccgatttcggcgggcatggcaccatttggaagctcttcctccggttccagcagaacctgcta

SEQ ID NO: 46 - protein, 22 aa, Homo sapiens
HADFGGHGTIWKLFLRFQQNLL

SEQ ID NO: 47 - DNA, 36 bp, Homo sapiens
  source 1..36: mol_type = genomic DNA
ctgcataccctgctggacctgcaagtattcggcaac

SEQ ID NO: 48 - protein, 12 aa, Homo sapiens
LHTLLDLQVFGN

SEQ ID NO: 49 - DNA, 27 bp, Homo sapiens
  source 1..27: mol_type = genomic DNA
gaggttagccagcatctagactatgcc

SEQ ID NO: 50 - protein, 9 aa, Homo sapiens
EVSQHLDYA

SEQ ID NO: 51 - DNA, 28 bp, synthetic construct
  misc_feature 1..28: note = Optimized RSS
  source 1..28: mol_type = other DNA
  variation 10..21: note = n is a, c, g or t
acaaaaaccnnnnnnnnnnnncacagtg

SEQ ID NO: 52 - DNA, 28 bp, synthetic construct
  misc_feature 1..28: note = Optimized RSS
  source 1..28: mol_type = other DNA
  variation 8..19: note = n is a, c, g or t
cacagtgnnnnnnnnnnnnacaaaaacc

SEQ ID NO: 53 - DNA, 28 bp, synthetic construct
  misc_feature 1..28: note = Optimized RSS
  source 1..28: mol_type = other DNA
  variation 10..21: note = n is a, c, g or t
  variation 3: note = w is a or t
  variation 5: note = w is a or t
  variation 9: note = w is a or t
  variation 6: note = y is c or t
ggwtwytgwnnnnnnnnnnnncactgtg

SEQ ID NO: 54 - DNA, 28 bp, synthetic construct
  misc_feature 1..28: note = Optimized RSS
  source 1..28: mol_type = other DNA
  variation 8..19: note = n is a, c, g or t
  variation 20: note = b is c, g or t
  variation 23: note = r is a or g
  variation 22: note = m is a or c
  variation 24: note = m is a or c
  variation 28: note = y is c or t
cacagtgnnnnnnnnnnnnbcmrmaacy

SEQ ID NO: 55 - DNA, 28 bp, synthetic construct
  misc_feature 1..28: note = Optimized RSS
  source 1..28: mol_type = other DNA
  variation 10..21: note = n is a, c, g or t
gatttttgtnnnnnnnnnnnntactgtg

SEQ ID NO: 56 - DNA, 28 bp, synthetic construct
  misc_feature 1..28: note = Optimized RSS
  source 1..28: mol_type = other DNA
  variation 8..19: note = n is a, c, g or t
cacagtgnnnnnnnnnnnnacaaaaacc

SEQ ID NO: 57 - DNA, 28 bp, synthetic construct
  misc_feature 1..28: note = Optimized RSS
  source 1..28: mol_type = other DNA
  variation 10..21: note = n is a, c, g or t
ggattttgtnnnnnnnnnnnncactgtg

SEQ ID NO: 58 - DNA, 28 bp, synthetic construct
  misc_feature 1..28: note = Optimized RSS
  source 1..28: mol_type = other DNA
  variation 8..19: note = n is a, c, g or t
cacagtgnnnnnnnnnnnntcaaaaacc

SEQ ID NO: 59 - DNA, 28 bp, synthetic construct
  misc_feature 1..28: note = Optimized RSS
  source 1..28: mol_type = other DNA
ggattttgtacagccccgagtcactgtg

SEQ ID NO: 60 - DNA, 28 bp, synthetic construct
  misc_feature 1..28: note = Optimized RSS
  source 1..28: mol_type = other DNA
cacagtgagaaaaactgtgtcaaaaacc

SEQ ID NO: 61 - DNA, 28 bp, synthetic construct
  misc_feature 1..28: note = Optimized RSS
  source 1..28: mol_type = other DNA
ggattttgtacagccccgagtcactgtg

SEQ ID NO: 62 - DNA, 28 bp, synthetic construct
  misc_feature 1..28: note = Optimized RSS
  source 1..28: mol_type = other DNA
cacagtgagaaaagcttcgtcaaaaacc

SEQ ID NO: 63 - DNA, 28 bp, synthetic construct
  misc_feature 1..28: note = Optimized RSS
  source 1..28: mol_type = other DNA
ggattttgtacagccccgagtcactgtg

SEQ ID NO: 64 - DNA, 28 bp, synthetic construct
  misc_feature 1..28: note = Optimized RSS
  source 1..28: mol_type = other DNA
cacagtgagaatagctacgtcaaaaacc

SEQ ID NO: 65 - DNA, 28 bp, synthetic construct
  misc_feature 1..28: note = Optimized RSS
  source 1..28: mol_type = other DNA
ggattttgtacagccccgagtcactgtg

SEQ ID NO: 66 - DNA, 28 bp, synthetic construct
  misc_feature 1..28: note = Optimized RSS
  source 1..28: mol_type = other DNA
cacagtgagaaaaactgtgtcaaaaacc

SEQ ID NO: 67 - DNA, 28 bp, synthetic construct
  misc_feature 1..28: note = Optimized RSS
  source 1..28: mol_type = other DNA
ggattttgtacagccccgagtcactgtg

SEQ ID NO: 68 - DNA, 28 bp, synthetic construct
  misc_feature 1..28: note = Optimized RSS
  source 1..28: mol_type = other DNA
cacagtgagaaaagctatgtcaaaaacc

SEQ ID NO: 69 - DNA, 28 bp, synthetic construct
  misc_feature 1..28: note = Optimized RSS
  source 1..28: mol_type = other DNA
ggattttgtgggggctcgtgtcactgtg

SEQ ID NO: 70 - DNA, 28 bp, synthetic construct
  misc_feature 1..28: note = Optimized RSS
  source 1..28: mol_type = other DNA
cacagtgacacagccccattcaaaaacc

SEQ ID NO: 71 - DNA, 28 bp, synthetic construct
  misc_feature 1..28: note = Optimized RSS
  source 1..28: mol_type = other DNA
ggattttgtgggggctcgtgtcactgtg

SEQ ID NO: 72 - DNA, 28 bp, synthetic construct
  misc_feature 1..28: note = optimized RSS
  source 1..28: mol_type = other DNA
cacagtgacacagccccattcaaaaacc

SEQ ID NO: 73 - DNA, 28 bp, synthetic construct
  misc_feature 1..28: note = Optimized RSS
  source 1..28: mol_type = other DNA
ggattttgtgggggctcgtgtcactgtg

SEQ ID NO: 74 - DNA, 28 bp, synthetic construct
  misc_feature 1..28: note = Optimized RSS
  source 1..28: mol_type = other DNA
cacagtgacacagacccattcaaaaacc

SEQ ID NO: 75 - DNA, 28 bp, synthetic construct
  misc_feature 1..28: note = Optimized RSS
  source 1..28: mol_type = other DNA
ggattttgtgggggttcgtgtcactgtg

SEQ ID NO: 76 - DNA, 28 bp, synthetic construct
  misc_feature 1..28: note = Optimized RSS
  source 1..28: mol_type = other DNA
cacagtgacacaaccccattcaaaaacc

SEQ ID NO: 77 - DNA, 28 bp, synthetic construct
  misc_feature 1..28: note = Optimized RSS
  source 1..28: mol_type = other DNA
ggattttgttgaggtctgtgtcactgtg

SEQ ID NO: 78 - DNA, 28 bp, synthetic construct
  misc_feature 1..28: note = Optimized RSS
  source 1..28: mol_type = other DNA
cacagtgtcacagagtccatcaaaaacc

SEQ ID NO: 79 - DNA, 28 bp, synthetic construct
  misc_feature 1..28: note = Optimized RSS
  source 1..28: mol_type = other DNA
ggattttgttgaggtctgtgtcactgtg

SEQ ID NO: 80 - DNA, 28 bp, synthetic construct
  misc_feature 1..28: note = Optimized RSS
  source 1..28: mol_type = other DNA
cacagtgtcacagagtccatcaaaaacc

SEQ ID NO: 81 - DNA, 28 bp, synthetic construct
  misc_feature 1..28: note = Optimized RSS
  source 1..28: mol_type = other DNA
ggattttgttgaggtctgtgtcactgtg

SEQ ID NO: 82 - DNA, 28 bp, synthetic construct
  misc_feature 1..28: note = Optimized RSS
  source 1..28: mol_type = other DNA
cacagtgtcacagagtccatcaaaaacc

SEQ ID NO: 83 - DNA, 28 bp, synthetic construct
  misc_feature 1..28: note = Optimized RSS
  source 1..28: mol_type = other DNA
ggattttgttgaggtctgtgtcactgtg

SEQ ID NO: 84 - DNA, 28 bp, synthetic construct
  misc_feature 1..28: note = Optimized RSS
  source 1..28: mol_type = other DNA
cacagtgtcacacggtccatcaaaaacc

SEQ ID NO: 85 - DNA, 28 bp, synthetic construct
  misc_feature 1..28: note = Optimized RSS
  source 1..28: mol_type = other DNA
ggattttgttgaggtctgtgtcactgtg

SEQ ID NO: 86 - DNA, 28 bp, synthetic construct
  misc_feature 1..28: note = Optimized RSS
  source 1..28: mol_type = other DNA
cacagtgtcacagagtccatcaaaaacc

SEQ ID NO: 87 - DNA, 28 bp, synthetic construct
  misc_feature 1..28: note = Optimized RSS
  source 1..28: mol_type = other DNA
ggattttgtgaagggtcctcccactgtg

SEQ ID NO: 88 - DNA, 28 bp, synthetic construct
  misc_feature 1..28: note = Optimized RSS
  source 1..28: mol_type = other DNA
cacagtgatgaacccagcatcaaaaacc

SEQ ID NO: 89 - DNA, 28 bp, synthetic construct
  misc_feature 1..28: note = Optimized RSS
  source 1..28: mol_type = other DNA
ggattttgtgaagggccctcccactgtg

SEQ ID NO: 90 - DNA, 28 bp, synthetic construct
  misc_feature 1..28: note = Optimized RSS
  source 1..28: mol_type = other DNA
cacagtgatgaacccagtgtcaaaaacc

SEQ ID NO: 91 - DNA, 28 bp, synthetic construct
  misc_feature 1..28: note = Optimized RSS
  source 1..28: mol_type = other DNA
ggattttgtgaaggcccctcccactgtg

SEQ ID NO: 92 - DNA, 28 bp, synthetic construct
  misc_feature 1..28: note = Optimized RSS
  source 1..28: mol_type = other DNA
cacagtgatgaaactagcatcaaaaacc

SEQ ID NO: 93 - DNA, 28 bp, synthetic construct
  misc_feature 1..28: note = Optimized RSS
  source 1..28: mol_type = other DNA
ggattttgtgaagggccctcccactgtg

SEQ ID NO: 94 - DNA, 28 bp, synthetic construct
  misc_feature 1..28: note = Optimized RSS
  source 1..28: mol_type = other DNA
cacagtgatgaaaccagcatcaaaaacc

SEQ ID NO: 95 - DNA, 28 bp, synthetic construct
  misc_feature 1..28: note = Optimized RSS
  source 1..28: mol_type = other DNA
ggattttgtcagggggtgtcacactgtg

SEQ ID NO: 96 - DNA, 28 bp, synthetic construct
  misc_feature 1..28: note = Optimized RSS
  source 1..28: mol_type = other DNA
cacagtggtgctgcccatatcaaaaacc

SEQ ID NO: 97 - DNA, 28 bp, synthetic construct
  misc_feature 1..28: note = Optimized RSS
  source 1..28: mol_type = other DNA
ggattttgtcaggcgatgtcacactgtg

SEQ ID NO: 98 - DNA, 28 bp, synthetic construct
  misc_feature 1..28: note = Optimized RSS
  source 1..28: mol_type = other DNA
cacagtggtgccgcccatatcaaaaacc

SEQ ID NO: 99 - DNA, 28 bp, synthetic construct
  misc_feature 1..28: note = Optimized RSS
  source 1..28: mol_type = other DNA
ggattttgtcagggggtgtcacactgtg

SEQ ID NO: 100 - DNA, 28 bp, synthetic construct
  misc_feature 1..28: note = Optimized RSS
  source 1..28: mol_type = other DNA
cacagtggtgctgcccatatcaaaaacc

SEQ ID NO: 101 - DNA, 28 bp, synthetic construct
  misc_feature 1..28: note = Optimized RSS
  source 1..28: mol_type = other DNA
ggattttgtcagggggtgccacactgtg

SEQ ID NO: 102 - DNA, 28 bp, synthetic construct
  misc_feature 1..28: note = Optimized RSS
  source 1..28: mol_type = other DNA
cacagtggtgccgcccatatcaaaaacc

SEQ ID NO: 103 - DNA, 28 bp, synthetic construct
  misc_feature 1..28: note = Optimized RSS
  source 1..28: mol_type = other DNA
ggattttgtaggtgtctgtgtcactgtg

SEQ ID NO: 104 - DNA, 28 bp, synthetic construct
  misc_feature 1..28: note = Optimized RSS
  source 1..28: mol_type = other DNA
cacagtgacactcgccaggtcaaaaacc

SEQ ID NO: 105 - DNA, 28 bp, synthetic construct
  misc_feature 1..28: note = Optimized RSS
  source 1..28: mol_type = other DNA
ggattttgtaggtgtctgtgtcactgtg

SEQ ID NO: 106 - DNA, 28 bp, synthetic construct
  misc_feature 1..28: note = Optimized RSS
  source 1..28: mol_type = other DNA
cacagtgacactcacccagtcaaaaacc

SEQ ID NO: 107 - DNA, 28 bp, synthetic construct
  misc_feature 1..28: note = Optimized RSS
  source 1..28: mol_type = other DNA
ggattttgtagctgtctgtatcactgtg

SEQ ID NO: 108 - DNA, 28 bp, synthetic construct
  misc_feature 1..28: note = Optimized RSS
  source 1..28: mol_type = other DNA
cacagtgacactcgccaggtcaaaaacc

SEQ ID NO: 109 - DNA, 28 bp, synthetic construct
  misc_feature 1..28: note = Optimized RSS
  source 1..28: mol_type = other DNA
ggtttctgaagctgtctgtgtcacagtc

SEQ ID NO: 110 - DNA, 28 bp, synthetic construct
  misc_feature 1..28: note = Optimized RSS
  source 1..28: mol_type = other DNA
cacaatgacactgggcaggacagaaacc

SEQ ID NO: 111 - DNA, 28 bp, synthetic construct
  misc_feature 1..28: note = Optimized RSS
  source 1..28: mol_type = other DNA
gggtttggctgagctgagaaccactgtg

SEQ ID NO: 112 - DNA, 28 bp, synthetic construct
  misc_feature 1..28: note = Optimized RSS
  source 1..28: mol_type = other DNA
cacagtgattggcagctctacaaaaacc

SEQ ID NO: 113 - DNA, 20 bp, synthetic construct
  misc_feature 1..20: note = Primer and/or probe
  source 1..20: mol_type = other DNA
cacaggaaacagctatgacc

SEQ ID NO: 114 - DNA, 21 bp, synthetic construct
  misc_feature 1..21: note = Primer and/or probe
  source 1..21: mol_type = other DNA
ccagtgccctagagtcaccca

SEQ ID NO: 115 - DNA, 21 bp, synthetic construct
  misc_feature 1..21: note = Primer and/or probe
  source 1..21: mol_type = other DNA
ctcccactcatgatctataga

SEQ ID NO: 116 - DNA, 19 bp, synthetic construct
  misc_feature 1..19: note = Primer and/or probe
  source 1..19: mol_type = other DNA
ctggggctcgctttagttg

SEQ ID NO: 117 - DNA, 20 bp, synthetic construct
  misc_feature 1..20: note = Primer and/or probe
  source 1..20: mol_type = other DNA
tgatagccgttgtattcagc

SEQ ID NO: 118 - DNA, 21 bp, synthetic construct
  misc_feature 1..21: note = Primer and/or probe
  source 1..21: mol_type = other DNA
ccagtgccctagagtcaccca

SEQ ID NO: 119 - DNA, 20 bp, synthetic construct
  misc_feature 1..20: note = Primer and/or probe
  source 1..20: mol_type = other DNA
gccatttctgtctgcattcg

SEQ ID NO: 120 - DNA, 21 bp, synthetic construct
  misc_feature 1..21: note = Primer and/or probe
  source 1..21: mol_type = other DNA
ggttcatcatgccgtttgtga

SEQ ID NO: 121 - DNA, 20 bp, synthetic construct
  misc_feature 1..20: note = Primer and/or probe
  source 1..20: mol_type = other DNA
tgggctcgtagtttgacgtg

SEQ ID NO: 122 - DNA, 20 bp, synthetic construct
  misc_feature 1..20: note = Primer and/or probe
  source 1..20: mol_type = other DNA
ttacccacacttcacgcacg

SEQ ID NO: 123 - DNA, 19 bp, synthetic construct
  misc_feature 1..19: note = Primer and/or probe
  source 1..19: mol_type = other DNA
ttaaacgacgcctcgaatg

SEQ ID NO: 124 - DNA, 20 bp, synthetic construct
  misc_feature 1..20: note = Primer and/or probe
  source 1..20: mol_type = other DNA
gcaaccattcgttgtagtag

SEQ ID NO: 125 - DNA, 20 bp, synthetic construct
  misc_feature 1..20: note = Primer and/or probe
  source 1..20: mol_type = other DNA
ctaacgcagtcatgtaatgc

SEQ ID NO: 126 - DNA, 19 bp, synthetic construct
  misc_feature 1..19: note = Primer and/or probe
  source 1..19: mol_type = other DNA
gactgtcacccagcattac

SEQ ID NO: 127 - DNA, 20 bp, synthetic construct
  misc_feature 1..20: note = Primer and/or probe
  source 1..20: mol_type = other DNA
cgtcgcctctacgggaaatc

SEQ ID NO: 128 - DNA, 21 bp, synthetic construct
  misc_feature 1..21: note = Primer and/or probe
  source 1..21: mol_type = other DNA
ccagtgccctagagtcaccca

SEQ ID NO: 129 - DNA, 20 bp, synthetic construct
  misc_feature 1..20: note = Primer and/or probe
  source 1..20: mol_type = other DNA
gccatttctgtctgcattcg

SEQ ID NO: 130 - DNA, 22 bp, synthetic construct
  misc_feature 1..22: note = Primer and/or probe
  source 1..22: mol_type = other DNA
aaacaccacgtaggatttacgc

SEQ ID NO: 131 - DNA, 10213 bp, synthetic construct
  misc_feature 1..10213: note = D6-DH1166
  source 1..10213: mol_type = other DNA
tacgtagccgtttcgatcctcccgaattgactagtgggtaggcctggcggccgctgccatttcattacctctttctccgcacccgacatagataccggtggattcgaattctccccgttgaagctgacctgcccagaggggcctgggcccaccccacacaccggggcggaatgtgtacaggccccggtctctgtgggtgttccgctaactggggctcccagtgctcaccccacaactaaagcgagccccagcctccagagcccccgaaggagatgccgcccacaagcccagcccccatccaggaggccccagagctcagggcgccggggcggattttgtacagccccgagtcactgtgcggaaggatgctgtggttagctttggcaaagttttcctgccaccacagtgagaaaaactgtgtcaaaaaccgtctcctggcccctgctggaggccgcgccagagaggggagcagccgccccgaacctaggtcctgctcagctcacacgacccccagcacccagagcacaacggagtccccattgaatggtgaggacggggaccagggctccagggggtcatggaaggggctggaccccatcctactgctatggtcccagtgctcctggccagaactgaccctaccaccgacaagagtccctcagggaaacgggggtcactggcacctcccagcatcaaccccaggcagcacaggcataaaccccacatccagagccgactccaggagcagagacaccccagtaccctgggggacaccgaccctgatgactccccactggaatccaccccagagtccaccaggaccaaagaccccgcccctgtctctgtccctcactcaggacctgctgcggggcgggccatgagaccagactcgggcttagggaacaccactgtggccccaacctcgaccaggccacaggcccttccttcctgccctgcggcagcacagactttggggtctgtgcagagaggaatcacagaggccccaggctgaggtggtgggggtggaagacccccaggaggtggcccacttcccttcctcccagctggaacccaccatgaccttcttaagataggggtgtcatccgaggcaggtcctccatggagctcccttcaggctcctccccggtcctcactaggcctcagtcccggctgcgggaatgcagccaccacaggcacaccaggcagcccagacccagccagcctgcagtgcccaagcccacattctggagcagagcaggctgtgtctgggagagtctgggctccccaccgcccccccgcacaccccacccacccctgtccaggccctatgcaggagggtcagagccccccatggggtatggacttagggtctcactcacgtggctcccctcctgggtgaaggggtctcatgcccagatccccacagcagagctggtcaaaggtggaggcagtggccccagggccaccctgacctggaccctcaggctcctctagccctggctgccctgctgtccctgggaggcctggactccaccagaccacaggtccagggcaccgcccataggtgctgcccacactcagttcacaggaagaagataagctccagacccccaagactgggacctgccttcctgccaccgcttgtagctccagacctccgtgcctcccccgaccacttacacacgggccagggagctgttccacaaagatcaaccccaaaccgggaccgcctggcactcgggccgctgccacttccctctccatttgttcccagcacctctgtgctccctccctcctccctccttcaggggaacagcctgtgcagcccctccctgcaccccacaccctggggaggcccaaccctgcctccagccctttctcccccgctgctcttcctgcccatccagacaaccctggggtcccatccctgcagcctacaccctggtctccacccagacccctgtctctccctccagacacccctcccaggccaaccctgcacatgcaggccctccccttttctgctgccagagcctcagtttctaccctctgtgcctaccccctgcctcctcctgcccacaactcgagctcttcctctcctggggcccctgagccatggcactgaccgtgcactcccacccccacactgcccatgccctcaccttcctcctggacactctgaccccgctcccctcttggacccagccctggtatttccaggacaaaggctcacccaagtcttccccatgcaggcccttgccctcactgcccggttacacggcagcctcctgtgcacagaagcagggagctcagcccttccacaggcagaaggcactgaaagaaatcggcctccagcaccctgatgcacgtccgcctgtgtctctcactgcccgcacctgcagggaggctcggcactccctgtaaagacgagggatccaggcagcaacatcatgggagaatgcagggctcccagacagcccagccctctcgcaggcctctcctgggaagagacctgcagccaccactgaacagccacggagcccgctggatagtaactgagtcagtgaccgacctggagggcaggggagcagtgaaccggagcccagaccatagggacagagaccagccgctgacatcccgagcccctcactggcggccccagaacaccgcgtggaaacagaacagacccacattcccacctggaacagggcagacactgctgagcccccagcaccagccctgagaaacaccaggcaacggcatcagagggggctcctgagaaagaaaggaggggaggtctccttcaccagcaagtacttcccttgaccaaaaacagggtccacgcaactcccccaggacaaaggaggagccccctgtacagcactgggctcagagtcctctcccacacaccctgagtttcagacaaaaaccccctggaaatcatagtatcagcaggagaactagccagagacagcaagaggggactcagtgactcccgcggggacaggaggattttgtgggggctcgtgtcactgtgctgcataccctgctggacctgcaagtattcggcaactgtgaggttagccagcatctagactatgcccacagtgacacagccccattcaaaaacccctgctgtaaacgcttccacttctggagctgaggggctggggggagcgtctgggaagtagggcctaggggtggccatcaatgcccaaaacgcaccagactcccccccagacatcaccccactggccagtgagcagagtaaacagaaaatgagaagcagctgggaagcttgcacaggccccaaggaaagagctttggcgggtgtgcaagaggggatgcgggcagagcctgagcagggccttttgctgtttctgctttcctgtgcagatagttccataaactggtgttcaagatcgatggctgggagtgagcccaggaggacagtgtgggaagggcacagggaaggagaagcagccgctatcctacactgtcatctttcaagagtttgccctgtgcccacaatgctgcatcatgggatgcttaacagctgatgtagacacagctaaagagagaatcagtgaaatggatttgcagcacagatctgaataaattctccagaatgtggagccacacagaagcaagcacaaggaaagtgcctgatgcaagggcaaagtacagtgtgtaccttcaggctgggcacagacactctgaaaagccttggcaggaactccctgcaacaaagcagagccctgcaggcaatgccagctccagagccctccctgagagcctcatgggcaaagatgtgcacaacaggtgtttctcatagccccaaactgagaatgaagcaaacagccatctgaaggaaaacaggcaaataaacgatggcaggttcatgaaatgcaaacccagacagccagaaggacaacagtgagggttacaggtgactctgtggttgagttcatgacaatgctgagtaattggagtaacaaaggaaagtccaaaaaatactttcaatgtgatttcttctaaataaaatttacagccggcaaaatgaactatcttcttaagggataaactttccactaggaaaactataaggaaaatcaagaaaaggatgatcacataaacacagtggtcgttacttctactggggaaggaagagggtatgaactgagacacacagggttggcaagtctcctaacaagaacagaacaaatacattacagtaccttgaaaacagcagttaaaattctaaattgcaagaagaggaaaatgcacacagctgtgtttagaaaattctcagtccagcactgttcataatagcaaagacattaacccaggttggataaataaacgatgacacaggcaattgcacaatgatacagacatacattcagtatatgagacattgatgatgtatccccaaagaaatgactttaaagagaaaaggcctgatatgtggtggcactcacctccctgggcatccccggacaggctgcaggcacactgtgtggcagggcaggctggtacctgctggcagctcctggggcctgatgtggagcaggcacagagccgtatccccccgaggacatatacccccaaggacggcacagttggtacattccggagacaagcaactcagccacactcccaggccagagcccgagagggacgcccatgcacagggaggcagagcccagctcctccacagccagcagcacccgtgcaggggccgccatctggcaggcacagagcatgggctgggaggaggggcagggacaccaggcagggttggcaccaactgaaaattacagaagtctcatacatctacctcagccttgcctgacctgggcctcacctgacctggacctcacctggcctggacctcacctggcctagacctcacctctgggcttcacctgagctcggcctcacctgacttggaccttgcctgtcctgagctcacatgatctgggcctcacctgacctgggtttcacctgacctgggcttcacctgacctgggcctcatctgacctgggcctcactggcctggacctcacctggcctgggcttcacctggcctcaggcctcatctgcacctgctccaggtcttgctggaacctcagtagcactgaggctgcaggggctcatccagggttgcagaatgactctagaacctcccacatctcagctttctgggtggaggcacctggtggcccagggaatataaaaagcctgaatgatgcctgcgtgatttgggggcaatttataaacccaaaaggacatggccatgcagcgggtagggacaatacagacagatatcagcctgaaatggagcctcagggcacaggtgggcacggacactgtccacctaagccaggggcagacccgagtgtccccgcagtagacctgagagcgctgggcccacagcctcccctcggtgccctgctacctcctcaggtcagccctggacatcccgggtttccccaggcctggcggtaggattttgttgaggtctgtgtcactgtgcatggcagctactgccagcccgcagccactggctactgaggatgccgattctgagaatagcagcttctactactatgactacctggatgaagtagctttcatgctctgccggaaggatgctgtggttagctttggcaaagttttcctgccaccacagtgtcacagagtccatcaaaaacccatccctgggaaccttctgccacagccctccctgtggggcaccgccgcgtgccatgttaggattttgactgaggacacagcaccatgggtatggtggctaccgcagcagtgcagcccgtgacccaaacacacagggcagcaggcacaacagacaagcccacaagtgaccaccctgagctcctgcctgccagccctggagaccatgaaacagatggccaggattatcccataggtcagccagacctcagtccaacaggtctgcatcgctgctgccctccaataccagtccggatggggacagggctggcccacattaccatttgctgccatccggccaacagtcccagaagcccctccctcaaggctgggccacatgtgtggaccctgagagccccccatgtctgagtaggggcaccaggaaggtggggctggccctgtgcactgtccctgcccctgtggtccctggcctgcctggccctgacacctgggcctctcctgggtcatttccaagacagaagacattcccaggacagctggagctgggagtccatcatcctgcctggccgtcctgagtcctgcgcctttccaaacctcacccgggaagccaacagaggaatcacctcccacaggcagagacaaagaccttccagaaatctctgtctctctccccagtgggcaccctcttccagggcagtcctcagtgatatcacagtgggaacccacatctggatcgggactgcccccagaacacaagatggcccacagggacagccccacagcccagcccttcccagacccctaaaaggcgtcccaccccctgcatctgccccagggctcaaactccaggaggactgactcctgcacaccctcctgccagacatcacctcagcccctcctggaagggacaggagcgcgcaagggtgagtcagaccctcctgccctcgatggcaggcggagaagattcagaaaggtctgagatccccaggacgcagcaccactgtcaatgggggccccagacgcctggaccagggcctgcgtgggaaaggcctctgggcacactcagggggattttgtgaagggtcctcccactgtgcatggcagctactgccagcccgcagccactggctactgaggatgccgattctgagaatagcagcttctactactatgactacctggatgaagtagctttcatgctctgccggaaggatgctgtggttagctttggcaaagttttcctgccactgcataccctgctggacctgcaagtattcggcaactgtgaggttagccagcatctagactatgcccacagtgatgaacccagcatcaaaaaccgaccggactcccaaggtttatgcacacttctccgctcagagctctccaggatcagaagagccgggcccaagggtttctgcccagaccctcggcctctagggacatcttggccatgacagcccatgggctggtgccccacacatcgtctgccttcaaacaagggcttcagagggctctgaggtgacctcactgatgaccacaggtgccctggccccttccccaccagctgcaccagaccccgtcatgacagatgccccgattccaacagccaattcctggggccaggaatcgctgtagacaccagcctccttccaacacctcctgccaattgcctggattcccatcccggttggaatcaagaggacagcatcccccaggctcccaacaggcaggactcccacaccctcctctgagaggccgctgtgttccgtagggccaggctgcagacagtccccctcacctgccactagacaaatgcctgctgtagatgtccccacctggaaaataccactcatggagcccccagccccaggtacagctgtagagagagtctctgaggcccctaagaagtagccatgcccagttctgccgggaccctcggccaggctgacaggagtggacgctggagctgggcccatactgggccacataggagctcaccagtgagggcaggagagcacatgccggggagcacccagcctcctgctgaccagaggcccgtcccagagcccaggaggctgcagaggcctctccagggggacactgtgcatgtctggtccctgagcagccccccacgtccccagtcctgggggcccctggcacagctgtctggaccctctctattccctgggaagctcctcctgacagccccgcctccagttccaggtgtggattttgtcagggggtgtcacactgtgcagcttcttgtgcaagcacagtggtgctgcccatatcaaaaaccaggccaagtagacaggcccctgctgtgcagccccaggcctccagctcacctgcttctcctggggctctcaaggctgctgttttctgcactctcccctctgtggggagggttccctcagtgggagatctgttctcaacatcccacggcctcattcctgcaaggaaggccaatggatgggcaacctcacatgccgcggctaagatagggtgggcagcctggcggggacaggacatcctgctggggtatctgtcactgtgcctagtggggcactggctcccaaacaacgcagtccttgccaaaatccccacggcctcccccgctaggggctggcctgatctcctgcagtcctaggaggctgctgacctccagaatggctccgtccccagttccagggcgagagcagatcccaggccggctgcagactgggaggccaccccctccttcccagggttcactgcaggtgaccagggcaggaaatggcctgaacacagggataaccgggccatcccccaacagagtccaccccctcctgctctgtaccccgcaccccccaggccagcccatgacatccgacaaccccacaccagagtcactgcccggtgctgccctagggaggacccctcagcccccaccctgtctagaggactggggaggacaggacacgccctctccttatggttcccccacctggctctggctgggacccttggggtgtggacagaaaggacgcttgcctgattggcccccaggagcccagaacttctctccagggaccccagcccgagcacccccttacccaggacccagccctgcccctcctcccctctgctctcctctcatcaccccatgggaatccagaatccccaggaagccatcaggaagggctgagggaggaagtggggccactgcaccaccaggcaggaggctctgtctttgtgaacccagggaggtgccagcctcctagagggtatggtccaccctgcctatggctcccacagtggcaggctgcagggaaggaccagggacggtgtgggggagggctcagggccccgcgggtgctccatcttggatgagcctatctctctcacccacggactcgcccacctcctcttcaccctggccacacgtcgtccacaccatcctaagtcccacctacaccagagccggcacagccagtgcagacagaggctggggtgcaggggggccgactgggcagcttcggggagggaggaatggaggaaggggagttcagtgaagaggcccccctcccctgggtccaggatcctcctctgggacccccggatcccatcccctccaggctctgggaggagaagcaggatgggagaatctgtgcgggaccctctcacagtggaatacctccacagcggctcaggccagatacaaaagcccctcagtgagccctccactgcagtgctgggcctgggggcagccgctcccacacaggatgaacccagcaccccgaggatgtcctgccagggggagctcagagccatgaaggagcaggatatgggacccccgatacaggcacagacctcagctccattcaggactgccacgtcctgccctgggaggaacccctttctctagtccctgcaggccaggaggcagctgactcctgacttggacgcctattccagacaccagacagaggggcaggccccccagaaccagggatgaggacgccccgtcaaggccagaaaagaccaagttgcgctgagcccagcaagggaaggtccccaaacaaaccaggaggattttgtaggtgtctgtgtcactgtgcaaacccatgaaaaccccaagggagtttggaactgccatgccgatttcggcgggcatggcaccatttggaagctcttcctccggttccagcagaacctgctaccacagtgacactcgccaggtcaaaaaccccatcccaagtcagcggaatgcagagagagcagggaggacatgtttaggatctgaggccgcacctgacacccaggccagcagacgtctcctgtccacggcaccctgccatgtcctgcatttctggaagaacaagggcaggctgaagggggtccaggaccaggagatgggtccgctctacccagagaaggagccaggcaggacacaagcccccacgcgtgggctcgtagtttgacgtgcgtgaagtgtgggtaagaaagtacgta

SEQ ID NO: 132 - DNA, 9828 bp, synthetic construct
  misc_feature 1..9828: note = D6-D17613
  source 1..9828: mol_type = other DNA
gcggccgctgccatttcattacctctttctccgcacccgacatagattacgtaacgcgtgggctcgtagtttgacgtgcgtgaagtgtgggtaagaaagtccccattgaggctgacctgcccagagggtcctgggcccacccaacacaccggggcggaatgtgtgcaggcctcggtctctgtgggtgttccgctagctggggctcacagtgctcaccccacacctaaaacgagccacagcctccggagcccctgaaggagaccccgcccacaagcccagcccccacccaggaggccccagagcacagggcgccccgtcggattttgtacagccccgagtcactgtgcagcttcttgcacagtgagaaaagcttcgtcaaaaaccgtctcctggccacagtcggaggccccgccagagaggggagcagccaccccaaacccatgttctgccggctcccatgaccccgtgcacctggagccccacggtgtccccactggatgggaggacaagggccgggggctccggcgggtcggggcaggggcttgatggcttccttctgccgtggccccattgcccctggctggagttgacccttctgacaagtgtcctcagagagtcagggatcagtggcacctcccaacatcaaccccacgcagcccaggcacaaaccccacatccagggccaactccaggaacagagacaccccaataccctgggggaccccgaccctgatgactcccgtcccatctctgtccctcacttggggcctgctgcggggcgagcacttgggagcaaactcaggcttaggggacaccactgtgggcctgacctcgagcaggccacagacccttccctcctgccctggtgcagcacagactttggggtctgggcagggaggaacttctggcaggtcaccaagcacagagcccccaggctgaggtggccccagggggaaccccagcaggtggcccactacccttcctcccagctggaccccatgtcttccccaagataggggtgccatccaaggcaggtcctccatggagcccccttcaggctcctctccagaccccactgggcctcagtccccactctaggaatgcagccaccacgggcacaccaggcagcccaggcccagccaccctgcagtgcccaagcccacaccctggaggagagcagggtgcgtctgggaggggctgggctccccacccccacccccacctgcacaccccacccacccttgcccgggccccctgcaggagggtcagagcccccatgggatatggacttagggtctcactcacgcacctcccctcctgggagaaggggtctcatgcccagatccccccagcagcgctggtcacaggtagaggcagtggccccagggccaccctgacctggcccctcaggctcctctagccctggctgccctgctgtccctgggaggcctgggctccaccagaccacaggtctagggcaccgcccacactggggccgcccacacacagctcacaggaagaagataagctccagacccccaggcccgggacctgccttgctgctacgacttcctgccccagacctcgttgccctcccccgtccacttacacacaggccaggaagctgttcccacacagaccaaccccagacggggaccacctggcactcaggtcactgccatttccttctccattcacttccaatgcctctgtgcttcctccctcctccttccttcgggggagcaccctgtgcagctcctccctgcagtccacaccctggggagacccgaccctgcagcccacaccctggggagacctgaccctcctccagccctttctcccccgctgctcttgccacccaccaagacagccctggggtcctgtccctacagcccccacccagttctctacctagacccgtcttcctccctctaaacacctctcccaggccaaccctacacctgcaggccctcccctccactgccaaagaccctcagtttctcctgcctgtgcccacccccgtgctcctcctgcccacagctcgagctcttcctctcctagggcccctgagggatggcattgaccgtgccctcgcacccacacactgcccatgccctcacattcctcctggccactccagccccactcccctctcaggcctggctctggtatttctgggacaaagccttacccaagtctttcccatgcaggcctgggcccttaccctcactgcccggttacagggcagcctcctgtgcacagaagcagggagctcagcccttccacaggcagaaggcactgaaagaaatcggcctccagcgccttgacacacgtctgcctgtgtctctcactgcccgcacctgcagggaggctcggcactccctctaaagacgagggatccaggcagcagcatcacaggagaatgcagggctaccagacatcccagtcctctcacaggcctctcctgggaagagacctgaagacgcccagtcaacggagtctaacaccaaacctccctggaggccgatgggtagtaacggagtcattgccagacctggaggcaggggagcagtgagcccgagcccacaccatagggccagaggacagccactgacatcccaagccactcactggtggtcccacaacaccccatggaaagaggacagacccacagtcccacctggaccagggcagagactgctgagacccagcaccagaaccaaccaagaaacaccaggcaacagcatcagagggggctctggcagaacagaggaggggaggtctccttcaccagcaggcgcttcccttgaccgaagacaggatccatgcaactcccccaggacaaaggaggagccccttgttcagcactgggctcagagtcctctccaagacacccagagtttcagacaaaaaccccctggaatgcacagtctcagcaggagagccagccagagccagcaagatggggctcagtgacacccgcagggacaggaggattttgtgggggctcgtgtcactgtgctgcataccctgctggacctgcaagtattcggcaacagtgaggttagccagcatctagactatgcccacagtgacacagccccattcaaaaacccctactgcaaacgcattccacttctggggctgaggggctgggggagcgtctgggaaatagggctcaggggtgtccatcaatgcccaaaacgcaccagactcccctccatacatcacacccaccagccagcgagcagagtaaacagaaaatgagaagcaagctggggaagcttgcacaggccccaaggaaagagctttggcgggtgtgtaagaggggatgcgggcagagcctgagcagggccttttgctgtttctgctttcctgtgcagagagttccataaactggtgttcgagatcaatggctgggagtgagcccaggaggacagcgtgggaagagcacagggaaggaggagcagccgctatcctacactgtcatctttcgaaagtttgccttgtgcccacactgctgcatcatgggatgcttaacagctgatgtagacacagctaaagagagaatcagtgagatggatttgcagcacagatctgaataaattctccagaatgtggagcagcacagaagcaagcacacagaaagtgcctgatgcaaggacaaagttcagtgggcaccttcaggcattgctgctgggcacagacactctgaaaagccctggcaggaactccctgtgacaaagcagaaccctcaggcaatgccagccccagagccctccctgagagcctcatgggcaaagatgtgcacaacaggtgtttctcatagccccaaactgagagcaaagcaaacgtccatctgaaggagaacaggcaaataaacgatggcaggttcatgaaatgcaaacccagacagccacaagcacaaaagtacagggttataagcgactctggttgagttcatgacaatgctgagtaattggagtaacaaagtaaactccaaaaaatactttcaatgtgatttcttctaaataaaatttacaccctgcaaaatgaactgtcttcttaagggatacatttcccagttagaaaaccataaagaaaaccaagaaaaggatgatcacataaacacagtggtggttacttctgctggggaaggaagagggtatgaactgagatacacagggtgggcaagtctcctaacaagaacagaacgaatacattacagtaccttgaaaacagcagttaaacttctaaattgcaagaagaggaaaatgcacacagttgtgtttagaaaattctcagtccagcactgttcataatagcaaagacattaacccaggtcggataaataagcgatgacacaggcaattgcacaatgatacagacatatatttagtatatgagacatcgatgatgtatccccaaataaacgactttaaagagataaagggctgatgtgtggtggcattcacctccctgggatccccggacaggttgcaggctcactgtgcagcagggcaggcgggtacctgctggcagttcctggggcctgatgtggagcaagcgcagggccatatatcccggaggacggcacagtcagtgaattccagagagaagcaactcagccacactccccaggcagagcccgagagggacgcccacgcacagggaggcagagcccagcacctccgcagccagcaccacctgcgcacgggccaccaccttgcaggcacagagtgggtgctgagaggaggggcagggacaccaggcagggtgagcacccagagaaaactgcagacgcctcacacatccacctcagcctcccctgacctggacctcactggcctgggcctcacttaacctgggcttcacctgaccttggcctcacctgacttggacctcgcctgtcccaagctttacctgacctgggcctcaactcacctgaacgtctcctgacctgggtttaacctgtcctggaactcacctggccttggcttcccctgacctggacctcatctggcctgggcttcacctggcctgggcctcacctgacctggacctcatctggcctggacctcacctggcctggacttcacctggcctgggcttcacctgacctggacctcacctggcctcgggcctcacctgcacctgctccaggtcttgctggagcctgagtagcactgagggtgcagaagctcatccagggttggggaatgactctagaagtctcccacatctgacctttctgggtggaggcagctggtggccctgggaatataaaaatctccagaatgatgactctgtgatttgtgggcaacttatgaacccgaaaggacatggccatggggtgggtagggacatagggacagatgccagcctgaggtggagcctcaggacacaggtgggcacggacactatccacataagcgagggatagacccgagtgtccccacagcagacctgagagcgctgggcccacagcctcccctcagagccctgctgcctcctccggtcagccctggacatcccaggtttccccaggcctggcggtaggattttgttgaggtctgtgtcactgtgcatggcagctactgccagcccgcagccactggctactgaggatgccgattctgagaatagcagcttctactactatgactacctggatgaagtagctttcatgctccacagtgtcacagagtccatcaaaaacccatgcctggaagcttcccgccacagccctccccatggggccctgctgcctcctcaggtcagccccggacatcccgggtttccccaggctgggcggtaggattttgttgaggtctgtgtcactgtgccaaacccatgaaaaccccaagggagtttggaacagccatgccgatttcggcgggcatggcaccatttggaagctcttcctccggttccagcagaacctgctacccacagtgtcacagagtccatcaaaaacccatccctgggagcctcccgccacagccctccctgcaggggaccggtacgtgccatgttaggattttgatcgaggagacagcaccatgggtatggtggctaccacagcagtgcagcctgtgacccaaacccgcagggcagcaggcacgatggacaggcccgtgactgaccacgctgggctccagcctgccagccctggagatcatgaaacagatggccaaggtcaccctacaggtcatccagatctggctccgaggggtctgcatcgctgctgccctcccaacgccagtccaaatgggacagggacggcctcacagcaccatctgctgccatcaggccagcgatcccagaagcccctccctcaaggctgggcacatgtgtggacactgagagccctcatatctgagtaggggcaccaggagggaggggctggccctgtgcactgtccctgcccctgtggtccctggcctgcctggccctgacacctgagcctctcctgggtcatttccaagacagaagacattcctggggacagccggagctgggcgtcgctcatcctgcccggccgtcctgagtcctgctcatttccagacctcaccggggaagccaacagaggactcgcctcccacattcagagacaaagaaccttccagaaatccctgcctctctccccagtggacaccctcttccaggacagtcctcagtggcatcacagcggcctgagatccccaggacgcagcaccgctgtcaataggggccccaaatgcctggaccagggcctgcgtgggaaaggcctctggccacactcggggattttgtgaagggccctcccactgtgccagcttcttgagccatgccgatttcggcgggcatggcaccatttggaagctcttcctccggttccagcagaacctgctaccacagtgatgaacccagtgtcaaaaaccggctggaaacccaggggctgtgtgcacgcctcagcttggagctctccaggagcacaagagccgggcccaaggatttgtgcccagaccctcagcctctagggacacctgggtcatctcagcctgggctggtgccctgcacaccatcttcctccaaataggggcttcagagggctctgaggtgacctcactcatgaccacaggtgacctggcccttccctgccagctataccagaccctgtcttgacagatgccccgattccaacagccaattcctgggaccctgaatagctgtagacaccagcctcattccagtacctcctgccaattgcctggattcccatcctggctggaatcaagaaggcagcatccgccaggctcccaacaggcaggactcccgcacaccctcctctgagaggccgctgtgttccgcagggccaggccctggacagttcccctcacctgccactagagaaacacctgccattgtcgtccccacctggaaaagaccactcgtggagcccccagccccaggtacagctgtagagacagtcctcgaggcccctaagaaggagccatgcccagttctgccgggaccctcggccaggccgacaggagtggacgctggagctgggcccacactgggccacataggagctcaccagtgagggcaggagagcacatgccggggagcacccagcctcctgctgaccagaggcccgtcccagagcccaggaggctgcagaggcctctccagggagacactgtgcatgtctggtacctaagcagccccccacgtccccagtcctgggggcccctggctcagctgtctgggccctccctgctccctgggaagctcctcctgacagccccgcctccagttccaggtgtggattttgtcaggcgatgtcacactgtgcagcttcttgagcaagcacagtggtgccgcccatatcaaaaaccaggccaagtagacaggcccctgctgcgcagccccaggcatccacttcacctgcttctcctggggctctcaaggctgctgtctgtcctctggccctctgtggggagggttccctcagtgggaggtctgtgctccagggcagggatgattgagatagaaatcaaaggctggcagggaaaggcagcttcccgccctgagaggtgcaggcagcaccacggagccacggagtcacagagccacggagcccccattgtgggcatttgagagtgctgtgcccccggcaggcccagccctgatggggaagcctgtcccatcccacagcccgggtcccacgggcagcgggcacagaagctgccaggttgtcctctatgatcctcatccctccagcagcatcccctccacagtggggaaactgaggcttggagcaccacccggccccctggaaatgaggctgtgagcccagacagtgggcccagagcactgtgagtaccccggcagtacctggctgcagggatcagccagagatgccaaaccctgagtgaccagcctacaggaggatccggccccacccaggccactcgattaatgctcaaccccctgccctggagacctcttccagtaccaccagcagctcagcttctcagggcctcatccctgcaaggaaggtcaagggctgggcctgccagaaacacagcaccctccctagccctggctaagacagggtgggcagacggctgtggacgggacatattgctggggcatttctcactgtcacttctgggtggtagctctgacaaaaacgcagaccctgccaaaatccccactgcctcccgctaggggctggcctggaatcctgctgtcctaggaggctgctgacctccaggatggctccgtccccagttccagggcgagagcagatcccaggcaggctgtaggctgggaggccacccctgcccttgccggggttgaatgcaggtgcccaaggcaggaaatggcatgagcacagggatgaccgggacatgccccaccagagtgcgccccttcctgctctgcaccctgcaccccccaggccagcccacgacgtccaacaactgggcctgggtggcagccccacccagacaggacagacccagcaccctgaggaggtcctgccagggggagctaagagccatgaaggagcaagatatggggcccccgatacaggcacagatgtcagctccatccaggaccacccagcccacaccctgagaggaacgtctgtctccagcctctgcaggtcgggaggcagctgacccctgacttggacccctattccagacaccagacagaggcgcaggccccccagaaccagggttgagggacgccccgtcaaagccagacaaaaccaaggggtgttgagcccagcaagggaaggcccccaaacagaccaggaggattttgtaggtgtctgtgtcactgtgcatggcagctactgccagcccgcagccactggctactgaggatgccgattctgagaatagcagcttctactactatgactacctggatgaagtagctttcatgctcagccggaaggatgctgtggttagctttggcaaagttttcctgccacccacagtgacactcacccagtcaaaaaccccattccaagtcagcggaagcagagagagcagggaggacacgtttaggatctgagactgcacctgacacccaggccagcagacgtctcccctccagggcaccccaccctgtcctgcatttctgcaagatcaggggcggcctgagggggggtctagggtgaggagatgggtcccctgtacaccaaggaggagttaggcaggtcccgagcactcttaattaaacgacgcctcgaatggaactactacaacgaatggttgctctacgtaatgcattcgctaccttaggaccgttatagttaggcgcgcc

SEQ ID NO: 133 - DNA, 9894 bp, synthetic construct
  misc_feature 1..9894: note = D6-DH114619
  source 1..9894: mol_type = other DNA
tacgtattaattaaacgacgcctcgaatggaactactacaacgaatggttgctctccccattgaggctgacctgcccagagagtcctgggcccaccccacacaccggggcggaatgtgtgcaggcctcggtctctgtgggtgttccgctagctggggctcacagtgctcaccccacacctaaaatgagccacagcctccggagcccccgcaggagaccccgcccacaagcccagcccccacccaggaggccccagagctcagggcgccccgtcggattttgtacagccccgagtcactgtgcaaacccatgaaaaccccaagggagtttggaaccacagtgagaatagctacgtcaaaaaccgtccagtggccactgccggaggccccgccagagagggcagcagccactctgatcccatgtcctgccggctcccatgacccccagcacgcggagccccacagtgtccccactggatgggaggacaagagctggggattccggcgggtcggggcaggggcttgatcgcatccttctgccgtggctccagtgcccctggctggagttgacccttctgacaagtgtcctcagagagacaggcatcaccggcgcctcccaacatcaaccccaggcagcacaggcacaaaccccacatccagagccaactccaggagcagagacaccccaataccctgggggaccccgaccctgatgacttcccactggaattcgccgtagagtccaccaggaccaaagaccctgcctctgcctctgtccctcactcaggacctgctgccgggcgaggccttgggagcagacttgggcttaggggacaccagtgtgaccccgaccttgaccaggacgcagacctttccttcctttcctggggcagcacagactttggggtctgggccaggaggaacttctggcaggtcgccaagcacagaggccacaggctgaggtggccctggaaagacctccaggaggtggccactccccttcctcccagctggaccccatgtcctccccaagataagggtgccatccaaggcaggtgctccttggagccccattcagactcctccctggaccccactgggcctcagtcccagctctggggatgaagccaccacaagcacaccaggcagcccaggcccagccaccctgcagtgcccaagcacacactctggagcagagcagggtgcctctgggaggggctgagctccccaccccacccccacctgcacaccccacccacccctgcccagcggctctgcaggagggtcagagccccacatggggtatggacttagggtctcactcacgtggctcccatcatgagtgaaggggcctcaagcccaggttcccacagcagcgcctgtcgcaagtggaggcagaggcccgagggccaccctgacctggtccctgaggttcctgcagcccaggctgccctgctgtccctgggaggcctgggctccaccagaccacaggtccagggcaccgggtgcaggagccacccacacacagctcacaggaagaagataagctccagacccccagggccagaacctgccttcctgctactgcttcctgccccagacctgggcgccctcccccgtccacttacacacaggccaggaagctgttcccacacagaacaaccccaaaccaggaccgcctggcactcaggtggctgccatttccttctccatttgctcccagcgcctctgtcctccctggttcctccttcgggggaacagcctgtgcagccagtccctgcagcccacaccctggggagacccaaccctgcctggggcccttccaaccctgctgctcttactgcccacccagaaaactctggggtcctgtccctgcagtccctaccctggtctccacccagacccctgtgtatcactccagacacccctcccaggcaaaccctgcacctgcaggccctgtcctcttctgtcgctagagcctcagtttctcccccctgtgcccacaccctacctcctcctgcccacaactctaactcttcttctcctggagcccctgagccatggcattgaccctgccctcccaccacccacagcccatgccctcaccttcctcctggccactccgaccccgccccctctcaggccaagccctggtatttccaggacaaaggctcacccaagtctttcccaggcaggcctgggctcttgccctcacttcccggttacacgggagcctcctgtgcacagaagcagggagctcagcccttccacaggcagaaggcactgaaagaaatcggcctccagcaccttgacacacgtccgcccgtgtctctcactgcccgcacctgcagggaggctccgcactccctctaaagacaagggatccaggcagcagcatcacgggagaatgcagggctcccagacatcccagtcctctcacaggcctctcctgggaagagacctgcagccaccaccaaacagccacagaggctgctggatagtaactgagtcaatgaccgacctggagggcaggggagcagtgagccggagcccataccatagggacagagaccagccgctgacatcccgagctcctcaatggtggccccataacacacctaggaaacataacacacccacagccccacctggaacagggcagagactgctgagcccccagcaccagccccaagaaacaccaggcaacagtatcagagggggctcccgagaaagagaggaggggagatctccttcaccatcaaatgcttcccttgaccaaaaacagggtccacgcaactcccccaggacaaaggaggagccccctatacagcactgggctcagagtcctctctgagacaccctgagtttcagacaacaacccgctggaatgcacagtctcagcaggagaacagaccaaagccagcaaaagggacctcggtgacaccagtagggacaggaggattttgtgggggctcgtgtcactgtgcaaacccatgaaaaccccaagggagtttggaactgcaagcacagtgacacagacccattcaaaaacccctactgcaaacacacccactcctggggctgaggggctgggggagcgtctgggaagtagggtccaggggtgtctatcaatgtccaaaatgcaccagactccccgccaaacaccaccccaccagccagcgagcagggtaaacagaaaatgagaggctctgggaagcttgcacaggccccaaggaaagagctttggcgggtgtgcaagaggggatgcaggcagagcctgagcagggccttttgctgtttctgctttcctgtgcagagagttccataaactggtgttcaagatcagtggctgggaatgagcccaggagggcagtctgtgggaagagcacagggaaggaggagcagccgctatcctacactgtcatctttcaaaagtttgccttgtgaccacactattgcatcatgggatgcttaagagctgatgtagacacagctaaagagagaatcagtgagatgaatttgcagcatagatctgaataaactctccagaatgtggagcagtacagaagcaaacacacagaaagtgcctgatgcaaggacaaagttcagtgggcaccttcaggcattgctgctgggcacagacactctgaaaagccttggcaggatctccctgcgacaaagcagaaccctcaggcaatgccagccccagagccctccctgagagcgtcatggggaaagatgtgcagaacagctgattatcatagactcaaactgagaacagagcaaacgtccatctgaagaacagtcaaataagcaatggtaggttcatgcaatgcaaacccagacagccaggggacaacagtagagggctacaggcggctttgcggttgagttcatgacaatgctgagtaattggagtaacagaggaaagcccaaaaaatacttttaatgtgatttcttctaaataaaatttacaccaggcaaaatgaactgtcttcttaagggataaactttcccctggaaaaactacaaggaaaattaagaaaacgatgatcacataaacacagttgtggttacttctactggggaaggaagagggtatgagctgagacacacagagtcggcaagtctccaagcaagcacagaacgaatacattacagtaccttgaatacagcagttaaacttctaaatcgcaagaacaggaaaatgcacacagctgtgtttagaaaattctcagtccagcactattcataatagcaaagacattaacccaggttggataaataaatgatgacacaggcaattgcacaatgatacagacatacatttagtacatgagacatcgatgatgtatccccaaagaaatgactttaaagagaaaaggcctgatgtgtggtggcactcacctccctgggatccccggacaggttgcaggcacactgtgtggcagggcaggctggtacatgctggcagctcctggggcctgatgtggagcaagcgcagggctgtatacccccaaggatggcacagtcagtgaattccagagagaagcagctcagccacactgcccaggcagagcccgagagggacgcccacgtacagggaggcagagcccagctcctccacagccaccaccacctgtgcacgggccaccaccttgcaggcacagagtgggtgctgagaggaggggcagggacaccaggcagggtgagcacccagagaaaactgcagaagcctcacacatccacctcagcctcccctgacctggacctcacctggtctggacctcacctggcctgggcctcacctgacctggacctcacctggcctgggcttcacctgacctggacctcacctggcctccggcctcacctgcacctgctccaggtcttgctggaacctgagtagcactgaggctgcagaagctcatccagggttggggaatgactctggaactctcccacatctgacctttctgggtggaggcatctggtggccctgggaatataaaaagccccagaatggtgcctgcgtgatttgggggcaatttatgaacccgaaaggacatggccatggggtgggtagggacatagggacagatgccagcctgaggtggagcctcaggacacagttggacgcggacactatccacataagcgagggacagacccgagtgttcctgcagtagacctgagagcgctgggcccacagcctcccctcggtgccctgctgcctcctcaggtcagccctggacatcccgggtttccccaggccagatggtaggattttgttgaggtctgtgtcactgtgcatggcagctactgccagcccgcagccactggctactgaggatgccgattctgagaatagcagcttctactactatgactacctggatgaagtagctttcatgctctgcgaggttagccagcatctagactatgcccacagtgtcacacggtccatcaaaaacccatgccacagccctccccgcaggggaccgccgcgtgccatgttacgattttgatcgaggacacagcgccatgggtatggtggctaccacagcagtgcagcccatgacccaaacacacagggcagcaggcacaatggacaggcctgtgagtgaccatgctgggctccagcccgccagccccggagaccatgaaacagatggccaaggtcaccccacagttcagccagacatggctccgtggggtctgcatcgctgctgccctctaacaccagcccagatggggacaaggccaaccccacattaccatctcctgctgtccacccagtggtcccagaagcccctccctcatggctgagccacatgtgtgaaccctgagagcaccccatgtcagagtaggggcagcagaagggcggggctggccctgtgcactgtccctgcacccatggtccctcgcctgcctggccctgacacctgagcctcttctgagtcatttctaagatagaagacattcccggggacagccggagctgggcgtcgctcatcccgcccggccgtcctgagtcctgcttgtttccagacctcaccagggaagccaacagaggactcacctcacacagtcagagacaaagaaccttccagaaatccctgtctcactccccagtgggcaccttcttccaggacattcctcggtcgcatcacagcaggcacccacatctggatcaggacggcccccagaacacaagatggcccatggggacagccccacaacccaggccttcccagacccctaaaaggcgtcccaccccctgcacctgccccagggctaaaaatccaggaggcttgactcccgcataccctccagccagacatcacctcagccccctcctggaggggacaggagcccgggagggtgagtcagacccacctgccctcgatggcaggcggggaagattcagaaaggcctgagatccccaggacgcagcaccactgtcaatgggggccccagacgcctggaccagggcctgcgtgggaaaggccgctgggcacactcagggggattttgtgaaggcccctcccactgtgcagcttcttgtgcaagcaaacccatgaaaaccccaagggagtttggaactgccatgccgatttcggcgggcatggcaccatttggaagctcttcctccggttccagcagaacctgctaccacagtgatgaaactagcatcaaaaaccggccggacacccagggaccatgcacacttctcagcttggagctctccaggaccagaagagtcaggtctgagggtttgtagccagaccctcggcctctagggacaccctggccatcacagcggatgggctggtgccccacatgccatctgctccaaacaggggcttcagagggctctgaggtgacttcactcatgaccacaggtgccctggccccttccccgccagctacaccgaaccctgtcccaacagctgccccagttccaacagccaattcctggggcccagaattgctgtagacaccagcctcgttccagcacctcctgccaattgcctggattcacatcctggctggaatcaagagggcagcatccgccaggctcccaacaggcaggactcccgcacaccctcctctgagaggccgctgtgttccgcagggccaggccctggacagttcccctcacctgccactagagaaacacctgccattgtcgtccccacctggaaaagaccactcgtggagcccccagccccaggtacagctgtagagagactccccgagggatctaagaaggagccatgcgcagttctgccgggaccctcggccaggccgacaggagtggacactggagctgggcccacactgggccacataggagctcaccagtgagggcaggagagcacatgccggggagcacccagcctcctgctgaccagaggcccgtcccagagcccaggaggctgcagaggcctctccagggggacactgtgcatgtctggtccctgagcagccccccacgtccccagtcctgggggcccctggcacagctgtctggaccctccctgttccctgggaagctcctcctgacagccccgcctccagttccaggtgtggattttgtcagggggtgtcacactgtgctgcataccctgctggacctgcaagtattcggcaactgtcggaaggatgctgtggttagctttggcaaagttttcctgccaccacagtggtgctgcccatatcaaaaaccaggccaagtagacaggcccctgctgtgcagccccaggcctccacttcacctgcttctcctggggctctcaaggtcactgttgtctgtactctgccctctgtggggagggttccctcagtgggaggtctgttctcaacatcccagggcctcatgtctgcacggaaggccaatggatgggcaacctcacatgccgcggctaagatagggtgggcagcctggcgggggacagtacatactgctggggtgtctgtcactgtgcctagtggggcactggctcccaaacaacgcagtcctcgccaaaatccccacagcctcccctgctaggggctggcctgatctcctgcagtcctaggaggctgctgacctccagaatgtctccgtccccagttccagggcgagagcagatcccaggccggctgcagactgggaggccaccccctccttcccagggttcactggaggtgaccaaggtaggaaatggccttaacacagggatgactgcgccatcccccaacagagtcagccccctcctgctctgtaccccgcaccccccaggccagtccacgaaaaccagggccccacatcagagtcactgcctggcccggccctggggcggacccctcagcccccaccctgtctagaggacttggggggacaggacacaggccctctccttatggttcccccacctgcctccggccgggacccttggggtgtggacagaaaggacacctgcctaattggcccccaggaacccagaacttctctccagggaccccagcccgagcacccccttacccaggacccagccctgcccctcctcccctctgctctcctctcatcaccccatgggaatccggtatccccaggaagccatcaggaagggctgaaggaggaagcggggccgtgcaccaccgggcaggaggctccgtcttcgtgaacccagggaagtgccagcctcctagagggtatggtccaccctgcctggggctcccaccgtggcaggctgcggggaaggaccagggacggtgtgggggagggctcagggccctgcgggtgctcctccatcttcggtgagcctcccccttcacccaccgtcccgcccacctcctctccaccctggctgcacgtcttccacaccatcctgagtcctacctacaccagagccagcaaagccagtgcagacaaaggctggggtgcaggggggctgccagggcagcttcggggagggaaggatggagggaggggaggtcagtgaagaggcccccttcccctgggtccaggatcctcctctgggacccccggatcccatcccctcctggctctgggaggagaagcaggatgggagaatctgtgcgggaccctctcacagtggaatatccccacagcggctcaggccagacccaaaagcccctcagtgagccctccactgcagtcctgggcctgggtagcagcccctcccacagaggacagacccagcaccccgaagaagtcctgccagggggagctcagagccatgaaagagcaggatatggggtccccgatacaggcacagacctcagctccatccaggcccaccgggacccaccatgggaggaacacctgtctccgggttgtgaggtagctggcctctgtctcggaccccactccagacaccagacagaggggcaggccccccaaaaccagggttgagggatgatccgtcaaggcagacaagaccaaggggcactgaccccagcaagggaaggctcccaaacagacgaggaggattttgtagctgtctgtatcactgtgcagcttcttgtgccatgccgatttcggcgggcatggcaccatttggaagctcttcctccggttccagcagaacctgctaccacagtgacactcgccaggtcaaaaaccccgtcccaagtcagcggaagcagagagagcagggaggacacgtttaggatctgaggccgcacctgacacccagggcagcagacgtctcccctccagggcaccctccaccgtcctgcgtttcttcaagaataggggcggcctgagggggtccagggccaggcgataggtcccctctaccccaaggaggagccaggcaggacccgagcaccgatgcatctaacgcagtcatgtaatgctgggtgacagtcagttcgcctacgta

SEQ ID NO: 134 - DNA, 11977 bp, synthetic construct
  misc_feature 1..11977: note = D6-DH120126
  source 1..11977: mol_type = other DNA
tacgtaatgcatctaacgcagtcatgtaatgctgggtgacagtcagttcgcctccccattgaggctgacctgcccagacgggcctgggcccaccccacacaccggggcggaatgtgtgcaggccccagtctctgtgggtgttccgctagctggggcccccagtgctcaccccacacctaaagcgagccccagcctccagagccccctaagcattccccgcccagcagcccagcccctgcccccacccaggaggccccagagctcagggcgcctggtcggattttgtacagccccgagtcactgtgcatgccgatttcggcgggcatggcaccatttggaagctcttcctccggttccagcagaacctgctaccacagtgagaaaaactgtgtcaaaaaccgactcctggcagcagtcggaggccccgccagagaggggagcagccggcctgaacccatgtcctgccggttcccatgacccccagcacccagagccccacggtgtccccgttggataatgaggacaagggctgggggctccggtggtttgcggcagggacttgatcacatccttctgctgtggccccattgcctctggctggagttgacccttctgacaagtgtcctcagaaagacagggatcaccggcacctcccaatatcaaccccaggcagcacagacacaaaccccacatccagagccaactccaggagcagagacaccccaacactctgggggaccccaaccgtgataactccccactggaatccgccccagagtctaccaggaccaaaggccctgccctgtctctgtccctcactcagggcctcctgcagggcgagcgcttgggagcagactcggtcttaggggacaccactgtgggccccaactttgatgaggccactgacccttccttcctttcctggggcagcacagactttggggtctgggcagggaagaactactggctggtggccaatcacagagcccccaggccgaggtggccccaagaaggccctcaggaggtggccactccacttcctcccagctggaccccaggtcctccccaagataggggtgccatccaaggcaggtcctccatggagcccccttcagactcctcccgggaccccactggacctcagtccctgctctgggaatgcagccaccacaagcacaccaggaagcccaggcccagccaccctgcagtgggcaagcccacactctggagcagagcagggtgcgtctgggaggggctaacctccccaccccccaccccccatctgcacacagccacctaccactgcccagaccctctgcaggagggccaagccaccatggggtatggacttagggtctcactcacgtgcctcccctcctgggagaaggggcctcatgcccagatccctgcagcactagacacagctggaggcagtggccccagggccaccctgacctggcatctaaggctgctccagcccagacagcactgccgttcctgggaagcctgggctccaccagaccacaggtccagggcacagcccacaggagccacccacacacagctcacaggaagaagataagctccagaccccagggcgggacctgccttcctgccaccacttacacacaggccagggagctgttcccacacagatcaaccccaaaccgggactgcctggcactagggtcactgccatttccctctccattccctcccagtgcctctgtgctccctccttctggggaacaccctgtgcagcccctccctgcagcccacacgctggggagaccccaccctgcctcgggccttttctacctgctgcacttgccgcccacccaaacaaccctgggtacgtgaccctgcagtcctcaccctgatctgcaaccagacccctgtccctccctctaaacacccctcccaggccaactctgcacctgcaggccctccgctcttctgccacaagagcctcaggttttcctacctgtgcccaccccctaacccctcctgcccacaacttgagttcttcctctcctggagcccttgagccatggcactgaccctacactcccacccacacactgcccatgccatcaccttcctcctggacactctgaccccgctcccctccctctcagacccggccctggtatttccaggacaaaggctcacccaagtcttccccatgcaggcccttgccctcactgcctggttacacgggagcctcctgtgcgcagaagcagggagctcagctcttccacaggcagaaggcactgaaagaaatcagcctccagtgccttgacacacgtccgcctgtgtctctcactgcctgcacctgcagggaggctccgcactccctctaaagatgagggatccaggcagcaacatcacgggagaatgcagggctcccagacagcccagccctctcgcaggcctctcctgggaagagacctgcagccaccactgaacagccacggaggtcgctggatagtaaccgagtcagtgaccgacctggagggcaggggagcagtgaaccggagcccataccatagggacagagaccagccgctaacatcccgagcccctcactggcggccccagaacaccccgtggaaagagaacagacccacagtcccacctggaacagggcagacactgctgagcccccagcaccagccccaagaaacactaggcaacagcatcagagggggctcctgagaaagagaggaggggaggtctccttcaccatcaaatgcttcccttgaccaaaaacagggtccacgcaactcccccaggacaaaggaggagccccctgtacagcactgggctcagagtcctctctgagacaggctcagtttcagacaacaacccgctggaatgcacagtctcagcaggagagccaggccagagccagcaagaggagactcggtgacaccagtctcctgtagggacaggaggattttgtgggggttcgtgtcactgtgcaaacccatgaaaaccccaagggagtttggaacagcaagcacagtgacacaaccccattcaaaaacccctactgcaaacgcacccactcctgggactgaggggctgggggagcgtctgggaagtatggcctaggggtgtccatcaatgcccaaaatgcaccagactctccccaagacatcaccccaccagccagtgagcagagtaaacagaaaatgagaagcagctgggaagcttgcacaggccccaaggaaagagctttggcaggtgtgcaagaggggatgtgggcagagcctcagcagggccttttgctgtttctgctttcctgtgcagagagttccataaactggtattcaagatcaatggctgggagtgagcccaggaggacagtgtgggaagagcacagggaaggaggagcagccgctatcctacactgtcatcttttgaaagtttgccctgtgcccacaatgctgcatcatgggatgcttaacagctgatgtagacacagctaaagagagaatcagtgaaatggatttgcagcacagatctgaataaatcctccagaatgtggagcagcacagaagcaagcacacagaaagtgcctgatgccaaggcaaagttcagtgggcaccttcaggcattgctgctgggcacagacactctgaaaagcactggcaggaactgcctgtgacaaagcagaaccctcaggcaatgccagccctagagcccttcctgagaacctcatgggcaaagatgtgcagaacagctgtttgtcatagccccaaactatggggctggacaaagcaaacgtccatctgaaggagaacagacaaataaacgatggcaggttcatgaaatgcaaactaggacagccagaggacaacagtagagagctacaggcggctttgcggttgagttcatgacaatgctgagtaattggagtaacagaggaaagcccaaaaaatacttttaatgtgatttcttctaaataaaatttacacccggcaaaatgaactatcttcttaagggataaactttcccctggaaaaactataaggaaaatcaagaaaacgatgatcacataaacacagtggtggttacttctactggggaaggaagagggtatgagctgagacacacagagtcggcaagtctcctaacaagaacagaacaaatacattacagtaccttgaaaacagcagttaaacttctaaatcgcaagaagaggaaaatgcacacacctgtgtttagaaaattctcagtccagcactgttcataatagcaaagacattaacccaggttggataaataagcgatgacacaggcaattgcacaatgatacagacatacattcagtatatgagacatcgatgatgtatccccaaagaaatgactttaaagagaaaaggcctgatgtgtggtggcaatcacctccctgggcatccccggacaggctgcaggctcactgtgtggcagggcaggcaggcacctgctggcagctcctggggcctgatgtggagcaggcacagagctgtatatccccaaggaaggtacagtcagtgcattccagagagaagcaactcagccacactccctggccagaacccaagatgcacacccatgcacagggaggcagagcccagcacctccgcagccaccaccacctgcgcacgggccaccaccttgcaggcacagagtgggtgctgagaggaggggcagggacaccaggcagggtgagcacccagagaaaactgcagaagcctcacacatccctcacctggcctgggcttcacctgacctggacctcacctggcctcgggcctcacctgcacctgctccaggtcttgctggagcctgagtagcactgaggctgtagggactcatccagggttggggaatgactctgcaactctcccacatctgacctttctgggtggaggcacctggtggcccagggaatataaaaagccccagaatgatgcctgtgtgatttgggggcaatttatgaacccgaaaggacatggccatggggtgggtagggacagtagggacagatgtcagcctgaggtgaagcctcaggacacaggtgggcatggacagtgtccacctaagcgagggacagacccgagtgtccctgcagtagacctgagagcgctgggcccacagcctcccctcggggccctgctgcctcctcaggtcagccctggacatcccgggtttccccaggcctggcggtaggattttgttgaggtctgtgtcactgtgcatggcagctactgccagcccgcagccactggctactgaggatgccgattctgagaatagcagcttctactactatgactacctggatgaagtagctttcatgctcagcgaggttagccagcatctagactatgcccacagtgtcacagagtccatcaaaaacccatgcctgggagcctcccaccacagccctccctgcgggggaccgctgcatgccgtgttaggattttgatcgaggacacggcgccatgggtatggtggctaccacagcagtgcagcccatgacccaaacacacggggcagcagaaacaatggacaggcccacaagtgaccatgatgggctccagcccaccagccccagagaccatgaaacagatggccaaggtcaccctacaggtcatccagatctggctccaaggggtctgcatcgctgctgccctcccaacgccaaaccagatggagacagggccggccccatagcaccatctgctgccgtccacccagcagtcccggaagcccctccctgaacgctgggccacgtgtgtgaaccctgcgagccccccatgtcagagtaggggcagcaggagggcggggctggccctgtgcactgtcactgcccctgtggtccctggcctgcctggccctgacacctgagcctctcctgggtcatttccaagacattcccagggacagccggagctgggagtcgctcatcctgcctggctgtcctgagtcctgctcatttccagacctcaccagggaagccaacagaggactcacctcacacagtcagagacaacgaaccttccagaaatccctgtttctctccccagtgagagaaaccctcttccagggtttctcttctctcccaccctcttccaggacagtcctcagcagcatcacagcgggaacgcacatctggatcaggacggcccccagaacacgcgatggcccatggggacagcccagcccttcccagacccctaaaaggtatccccaccttgcacctgccccagggctcaaactccaggaggcctgactcctgcacaccctcctgccagatatcacctcagccccctcctggaggggacaggagcccgggagggtgagtcagacccacctgccctcaatggcaggcggggaagattcagaaaggcctgagatccccaggacgcagcaccactgtcaatgggggccccagacgcctggaccagggcctgtgtgggaaaggcctctggccacactcagggggattttgtgaagggccctcccactgtggaggttagccagcatctagactatgcccacagtgatgaaaccagcatcaaaaaccgaccggactcgcagggtttatgcacacttctcggctcggagctctccaggagcacaagagccaggcccgagggtttgtgcccagaccctcggcctctagggacacccgggccatcttagccgatgggctgatgccctgcacaccgtgtgctgccaaacaggggcttcagagggctctgaggtgacttcactcatgaccacaggtgccctggtcccttcactgccagctgcaccagaccctgttccgagagatgccccagttccaaaagccaattcctggggccgggaattactgtagacaccagcctcattccagtacctcctgccaattgcctggattcccatcctggctggaatcaagagggcagcatccgccaggctcccaacaggcaggactcccacacaccctcctctgagaggccgctgtgttccgcagggccaggccgcagacagttcccctcacctgcccatgtagaaacacctgccattgtcgtccccacctggcaaagaccacttgtggagcccccagccccaggtacagctgtagagagagtcctcgaggcccctaagaaggagccatgcccagttctgccgggaccctcggccaggccgacaggagtggacgctggagctgggcccacactgggccacataggagctcaccagtgagggcaggagagcacatgccggggagcacccagcctcctgctgaccagagacccgtcccagagcccaggaggctgcagaggcctctccagggggacacagtgcatgtctggtccctgagcagcccccaggctctctagcactgggggcccctggcacagctgtctggaccctccctgttccctgggaagctcctcctgacagccccgcctccagttccaggtgtggattttgtcagggggtgccacactgtgctgcataccctgctggacctgcaagtattcggcaacagtcggaaggatgctgtggttagctttggcaaagttttcctgccaccacagtggtgccgcccatatcaaaaaccaggccaagtagacagacccctgccacgcagccccaggcctccagctcacctgcttctcctggggctctcaaggctgctgtctgccctctggccctctgtggggagggttccctcagtgggaggtctgtgctccagggcagggatgactgagatagaaatcaaaggctggcagggaaaggcagcttcccgccctgagaggtgcaggcagcaccacagagccatggagtcacagagccacggagcccccagtgtgggcgtgtgagggtgctgggctcccggcaggcccagccctgatggggaagcctgccccgtcccacagcccaggtccccaggggcagcaggcacagaagctgccaagctgtgctctacgatcctcatccctccagcagcatccactccacagtggggaaactgagccttggagaaccacccagccccctggaaacaaggcggggagcccagacagtgggcccagagcactgtgtgtatcctggcactaggtgcagggaccacccggagatccccatcactgagtggccagcctgcagaaggacccaaccccaaccaggccgcttgattaagctccatccccctgtcctgggaacctcttcccagcgccaccaacagctcggcttcccaggccctcatccctccaaggaaggccaaaggctgggcctgccaggggcacagtaccctcccttgccctggctaagacagggtgggcagacggctgcagataggacatattgctggggcatcttgctctgtgactactgggtactggctctcaacgcagaccctaccaaaatccccactgcctcccctgctaggggctggcctggtctcctcctgctgtcctaggaggctgctgacctccaggatggcttctgtccccagttctagggccagagcagatcccaggcaggctgtaggctgggaggccacccctgtccttgccgaggttcagtgcaggcacccaggacaggaaatggcctgaacacagggatgactgtgccatgccctacctaagtccgcccctttctactctgcaacccccactccccaggtcagcccatgacgaccaacaacccaacaccagagtcactgcctggccctgccctggggaggacccctcagcccccaccctgtctagaggagttggggggacaggacacaggctctctccttatggttcccccacctggctcctgccgggacccttggggtgtggacagaaaggacgcctgcctaattggcccccaggaacccagaacttctctccagggaccccagcccgagcacccccttacccaggacccagccctgcccctcctcccctctgctctcctctcatcactccatgggaatccagaatccccaggaagccatcaggaagggctgaaggaggaagcggggccgctgcaccaccgggcaggaggctccgtcttcgtgaacccagggaagtgccagcctcctagagggtatggtccaccctgcctggggctcccaccgtggcaggctgcggggaaggaccagggacggtgtgggggagggctcagggccctgcaggtgctccatcttggatgagcccatccctctcacccaccgacccgcccacctcctctccaccctggccacacgtcgtccacaccatcctgagtcccacctacaccagagccagcagagccagtgcagacagaggctggggtgcaggggggccgccagggcagctttggggagggaggaatggaggaaggggaggtcagtgaagaggcccccctcccctgggtctaggatccacctttgggacccccggatcccatcccctccaggctctgggaggagaagcaggatgggagattctgtgcaggaccctctcacagtggaatacctccacagcggctcaggccagatacaaaagcccctcagtgagccctccactgcagtgcagggcctgggggcagcccctcccacagaggacagacccagcaccccgaagaagtcctgccagggggagctcagagccatgaaggagcaagatatggggaccccaatactggcacagacctcagctccatccaggcccaccaggacccaccatgggtggaacacctgtctccggcccctgctggctgtgaggcagctggcctctgtctcggacccccattccagacaccagacagagggacaggccccccagaaccagtgttgagggacacccctgtccagggcagccaagtccaagaggcgcgctgagcccagcaagggaaggcccccaaacaaaccaggaggtttctgaagctgtctgtgtcacagtcgggcatagccacggctaccacaatgacactgggcaggacagaaaccccatcccaagtcagccgaaggcagagagagcaggcaggacacatttaggatctgaggccacacctgacactcaagccaacagatgtctcccctccagggcgccctgccctgttcagtgttcctgagaaaacaggggcagcctgaggggatccagggccaggagatgggtcccctctaccccgaggaggagccaggcgggaatcccagccccctccccattgaggccatcctgcccagaggggcccggacccaccccacacacccaggcagaatgtgtgcaggcctcaggctctgtgggtgccgctagctggggctgccagtcctcaccccacacctaaggtgagccacagccgccagagcctccacaggagaccccacccagcagcccagcccctacccaggaggccccagagctcagggcgcctgggtggattttgtacagccccgagtcactgtgctgcataccctgctggacctgcaagtattcggcaaccacagtgagaaaagctatgtcaaaaaccgtctcccggccactgctggaggcccagccagagaagggaccagccgcccgaacatacgaccttcccagacctcatgacccccagcacttggagctccacagtgtccccattggatggtgaggatgggggccggggccatctgcacctcccaacatcacccccaggcagcacaggcacaaaccccaaatccagagccgacaccaggaacacagacaccccaataccctgggggaccctggccctggtgacttcccactgggatccacccccgtgtccacctggatcaaagaccccaccgctgtctctgtccctcactcagggcctgctgaggggcgggtgctttggagcagactcaggtttaggggccaccattgtggggcccaacctcgaccaggacacagatttttctttcctgccctggggcaacacagactttggggtctgtgcagggaggaccttctggaaagtcaccaagcacagagccctgactgaggtggtctcaggaagacccccaggagggggcttgtgccccttcctctcatgtggaccccatgccccccaagataggggcatcatgcagggcaggtcctccatgcagccaccactaggcaactccctggcgccggtccccactgcgcctccatcccggctctggggatgcagccaccatggccacaccaggcagcccgggtccagcaaccctgcagtgcccaagcccttggcaggattcccagaggctggagcccacccctcctcatccccccacacctgcacacacacacctaccccctgcccagtccccctccaggagggttggagccgcccatagggtgggggctccaggtctcactcactcgcttcccttcctgggcaaaggagcctcgtgccccggtcccccctgacggcgctgggcacaggtgtgggtactgggccccagggctcctccagccccagctgccctgctctccctgggaggcctgggcaccaccagaccaccagtccagggcacagccccagggagccgcccactgccagctcacaggaagaagataagcttcagaccctcagggccgggagctgccttcctgccaccccttcctgccccagacctccatgccctcccccaaccacttacacacaagccagggagctgtttccacacagttcaaccccaaaccaggacggcctggcactcgggtcactgccatttctgtctgcattcgctcccagcgcccctgtgttccctccctcctccctccttcctttcttcctgcattgggttcatgccgcagagtgccaggtgcaggtcagccctgagcttggggtcacctcctcactgaaggcagcctcagggtgcccaggggcaggcagggtgggggtgaggcttccagctccaaccgcttcgctaccttaggaccgttatagttaggcgcgccgtcgaccaattctcatgtttgacagcttatcatcgaatttctacgta

SEQ ID NO: 135 - DNA, 17 bp, synthetic construct
  misc_feature 1..17: note = Primer and/or probe
  source 1..17: mol_type = other DNA
tgcggccgatcttagcc

SEQ ID NO: 136 - DNA, 21 bp, synthetic construct
  misc_feature 1..21: note = Primer and/or probe
  source 1..21: mol_type = other DNA
acgagcgggttcggcccattc

SEQ ID NO: 137 - DNA, 18 bp, synthetic construct
  misc_feature 1..18: note = Primer and/or probe
  source 1..18: mol_type = other DNA
ttgaccgattccttgcgg

SEQ ID NO: 138 - DNA, 19 bp, synthetic construct
  misc_feature 1..19: note = Primer and/or probe
  source 1..19: mol_type = other DNA
cgggtcactgccatttctg

SEQ ID NO: 139 - DNA, 20 bp, synthetic construct
  misc_feature 1..20: note = Primer and/or probe
  source 1..20: mol_type = other DNA
tctgcattcgctcccagcgc

SEQ ID NO: 140 - DNA, 19 bp, synthetic construct
  misc_feature 1..19: note = Primer and/or probe
  source 1..19: mol_type = other DNA
tctgcggcatgaacccaat

SEQ ID NO: 141 - DNA, 19 bp, synthetic construct
  misc_feature 1..19: note = Primer and/or probe
  source 1..19: mol_type = other DNA
tggccagaactgaccctac

SEQ ID NO: 142 - DNA, 20 bp, synthetic construct
  misc_feature 1..20: note = Primer and/or probe
  source 1..20: mol_type = other DNA
accgacaagagtccctcagg

SEQ ID NO: 143 - DNA, 19 bp, synthetic construct
  misc_feature 1..19: note = Primer and/or probe
  source 1..19: mol_type = other DNA
ggagtcggctctggatgtg

SEQ ID NO: 144 - DNA, 18 bp, synthetic construct
  misc_feature 1..18: note = Primer and/or probe
  source 1..18: mol_type = other DNA
ggagccaggcaggacaca

SEQ ID NO: 145 - DNA, 19 bp, synthetic construct
  misc_feature 1..19: note = Primer and/or probe
  source 1..19: mol_type = other DNA
tgggctcgtagtttgacgt

SEQ ID NO: 146 - DNA, 23 bp, synthetic construct
  misc_feature 1..23: note = Primer and/or probe
  source 1..23: mol_type = other DNA
gggactttcttacccacacttca

SEQ ID NO: 147 - DNA, 24 bp, synthetic construct
  misc_feature 1..24: note = Primer and/or probe
  source 1..24: mol_type = other DNA
ggtcccgagcactcttaattaaac

SEQ ID NO: 148 - DNA, 16 bp, synthetic construct
  misc_feature 1..16: note = Primer and/or probe
  source 1..16: mol_type = other DNA
cctcgaatggaactac

SEQ ID NO: 149 - DNA, 21 bp, synthetic construct
  misc_feature 1..21: note = Primer and/or probe
  source 1..21: mol_type = other DNA
gggagagcaaccattcgttgt

SEQ ID NO: 150 - DNA, 19 bp, synthetic construct
  misc_feature 1..19: note = Primer and/or probe
  source 1..19: mol_type = other DNA
ccgagcaccgatgcatcta

SEQ ID NO: 151 - DNA, 16 bp, synthetic construct
  misc_feature 1..16: note = Primer and/or probe
  source 1..16: mol_type = other DNA
cgcagtcatgtaatgc

SEQ ID NO: 152 - DNA, 20 bp, synthetic construct
  misc_feature 1..20: note = Primer and/or probe
  source 1..20: mol_type = other DNA
gggaggcgaactgactgtca

SEQ ID NO: 153 - DNA, 19 bp, synthetic construct
  misc_feature 1..19: note = Primer and/or probe
  source 1..19: mol_type = other DNA
ggtggagaggctattcggc

SEQ ID NO: 154 - DNA, 23 bp, synthetic construct
  misc_feature 1..23: note = Primer and/or probe
  source 1..23: mol_type = other DNA
tgggcacaacagacaatcggctg

SEQ ID NO: 155 - DNA, 17 bp, synthetic construct
  misc_feature 1..17: note = Primer and/or probe
  source 1..17: mol_type = other DNA
gaacacggcggcatcag

SEQ ID NO: 156 - DNA, 19 bp, synthetic construct
  misc_feature 1..19: note = Primer and/or probe
  source 1..19: mol_type = other DNA
cagtcccgttgatccagcc

SEQ ID NO: 157 - DNA, 30 bp, synthetic construct
  misc_feature 1..30: note = Primer and/or probe
  source 1..30: mol_type = other DNA
cccatcagggattttgtatctctgtggacg

SEQ ID NO: 158 - DNA, 21 bp, synthetic construct
  misc_feature 1..21: note = Primer and/or probe
  source 1..21: mol_type = other DNA
ggatatgcagcactgtgccac

SEQ ID NO: 159 - DNA, 19 bp, synthetic construct
  misc_feature 1..19: note = Primer and/or probe
  source 1..19: mol_type = other DNA
tcctccaacgacaggtccc

SEQ ID NO: 160 - DNA, 24 bp, synthetic construct
  misc_feature 1..24: note = Primer and/or probe
  source 1..24: mol_type = other DNA
tccctggaactctgccccgacaca

SEQ ID NO: 161 - DNA, 20 bp, synthetic construct
  misc_feature 1..20: note = Primer and/or probe
  source 1..20: mol_type = other DNA
gatgaactgacgggcacagg

SEQ ID NO: 162 - DNA, 20 bp, synthetic construct
  misc_feature 1..20: note = Primer and/or probe
  source 1..20: mol_type = other DNA
atcacactcatcccatcccc

SEQ ID NO: 163 - DNA, 29 bp, synthetic construct
  misc_feature 1..29: note = Primer and/or probe
  source 1..29: mol_type = other DNA
cccttccctaagtaccacagagtgggctc

SEQ ID NO: 164 - DNA, 20 bp, synthetic construct
  misc_feature 1..20: note = Primer and/or probe
  source 1..20: mol_type = other DNA
cacagggaagcaggaactgc

SEQ ID NO: 165 - DNA, 17 bp, synthetic construct
  misc_feature 1..17: note = Primer and/or probe
  source 1..17: mol_type = other DNA
gccatgcaaggccaagc

SEQ ID NO: 166 - DNA, 24 bp, synthetic construct
  misc_feature 1..24: note = Primer and/or probe
  source 1..24: mol_type = other DNA
ccaggaaaatgctgccagagcctg

SEQ ID NO: 167 - DNA, 24 bp, synthetic construct
  misc_feature 1..24: note = Primer and/or probe
  source 1..24: mol_type = other DNA
agttcttgagccttagggtgctag

SEQ ID NO: 168 - DNA, 20 bp, synthetic construct
  misc_feature 1..20: note = Primer and/or probe
  source 1..20: mol_type = other DNA
ccccacagcaaatcacaacc

SEQ ID NO: 169 - DNA, 27 bp, synthetic construct
  misc_feature 1..27: note = Primer and/or probe
  source 1..27: mol_type = other DNA
atgcagttgtcacccttgaggccattc

SEQ ID NO: 170 - DNA, 19 bp, synthetic construct
  misc_feature 1..19: note = Primer and/or probe
  source 1..19: mol_type = other DNA
tgtttcccaggcgtcactg

SEQ ID NO: 171 - DNA, 20 bp, synthetic construct
  misc_feature 1..20: note = Primer and/or probe
  source 1..20: mol_type = other DNA
ctcagtgattctggccctgc

SEQ ID NO: 172 - DNA, 32 bp, synthetic construct
  misc_feature 1..32: note = Primer and/or probe
  source 1..32: mol_type = other DNA
tgctccacagctacaaaccccttcctataatg

SEQ ID NO: 173 - DNA, 21 bp, synthetic construct
  misc_feature 1..21: note = Primer and/or probe
  source 1..21: mol_type = other DNA
ggatgatggctcagcacagag

SEQ ID NO: 174 - DNA, 20 bp, synthetic construct
  misc_feature 1..20: note = Primer and/or probe
  source 1..20: mol_type = other DNA
tggtcacctccaggagcctc

SEQ ID NO: 175 - DNA, 30 bp, synthetic construct
  misc_feature 1..30: note = Primer and/or probe
  source 1..30: mol_type = other DNA
agtctctgcttcccccttgtggctatgagc

SEQ ID NO: 176 - DNA, 21 bp, synthetic construct
  misc_feature 1..21: note = Primer and/or probe
  source 1..21: mol_type = other DNA
gctgcagggtgtatcaggtgc

SEQ ID NO: 177 - DNA, 18 bp, synthetic construct
  misc_feature 1..18: note = Primer and/or probe
  source 1..18: mol_type = other DNA
gtgtcacagtcgggcata

SEQ ID NO: 178 - DNA, 24 bp, synthetic construct
  misc_feature 1..24: note = Primer and/or probe
  source 1..24: mol_type = other DNA
ccacggctaccacaatgacactgg

SEQ ID NO: 179 - DNA, 20 bp, synthetic construct
  misc_feature 1..20: note = Primer and/or probe
  source 1..20: mol_type = other DNA
ccttcggctgacttgggatg

SEQ ID NO: 180 - DNA, 66 bp, synthetic construct
  misc_feature 1..66: note = mu-conotoxin or tarantula toxin ProTxII nucleic acid sequence
  source 1..66: mol_type = other DNA
gagagaagctgcaatggcagacgcggctgcagcagcagatggagccgcgatcatagcaggtgctgc

SEQ ID NO: 181 - protein, 22 aa, synthetic construct
  REGION 1..22: note = mu-conotoxin or tarantula toxin ProTxII amino acid sequence
ERSCNGRRGCSSRWSRDHSRCC

SEQ ID NO: 182 - DNA, 31 bp, synthetic construct
  misc_feature 1..31: note = mu-conotoxin or tarantula toxin ProTxII nucleic acid sequence
  source 1..31: mol_type = other DNA
aggatattgtagcagcagatggtgctatacc

SEQ ID NO: 183 - protein, 10 aa, synthetic construct
  REGION 1..10: note = mu-conotoxin or tarantula toxin ProTxII amino acid sequence
GYCSSRWCYT

SEQ ID NO: 184 - DNA, 58 bp, synthetic construct
  misc_feature 1..58: note = mu-conotoxin or tarantula toxin ProTxII nucleic acid sequence
  source 1..58: mol_type = other DNA
gtattacgattgcaactgcagcagatggcgcgaccatagcaggtgctgctattatacc

SEQ ID NO: 185 - protein, 19 aa, synthetic construct
  REGION 1..19: note = mu-conotoxin or tarantula toxin ProTxII amino acid sequence
YYDCNCSRWRDHSRCCYYT

SEQ ID NO: 186 - DNA, 66 bp, synthetic construct
  misc_feature 1..66: note = mu-conotoxin or tarantula toxin ProTxII nucleic acid sequence
  source 1..66: mol_type = other DNA
gagaggcttagctgtggcttccctaagagctgccgcagcaggcaaagcaagcctcacagatgctgc

SEQ ID NO: 187 - protein, 22 aa, synthetic construct
  REGION 1..22: note = mu-conotoxin or tarantula toxin ProTxII amino acid sequence
ERLSCGFPKSCRSRQSKPHRCC

SEQ ID NO: 188 - DNA, 90 bp, synthetic construct
  misc_feature 1..90: note = mu-conotoxin or tarantula toxin ProTxII nucleic acid sequence
  source 1..90: mol_type = other DNA
tacagccagaagtggatgtggacttgcgatagtgagaggaagtgcagtgagggtatggtatgccggctgtggtgtaagaagaagctctgg

SEQ ID NO: 189 - protein, 30 aa, synthetic construct
  REGION 1..30: note = mu-conotoxin or tarantula toxin ProTxII amino acid sequence
YSQKWMWTCDSERKCSEGMVCRLWCKKKLW

SEQ ID NO: 190 - DNA, 48 bp, synthetic construct
  misc_feature 1..48: note = mu-conotoxin or tarantula toxin ProTxII nucleic acid sequence
  source 1..48: mol_type = other DNA
agctgcaactgcagcagcaaatggagccgcgaccatagcaggtgctgc

SEQ ID NO: 191 - protein, 16 aa, synthetic construct
  REGION 1..16: note = mu-conotoxin or tarantula toxin ProTxII amino acid sequence
SCNCSSKWSRDHSRCC

SEQ ID NO: 192 - DNA, 57 bp, synthetic construct
  misc_feature 1..57: note = mu-conotoxin or tarantula toxin ProTxII nucleic acid sequence
  source 1..57: mol_type = other DNA
gagagatgcaatggcagacgcggctgcagcagatggcgcgatcatagcaggtgctgc

SEQ ID NO: 193 - protein, 19 aa, synthetic construct
  REGION 1..19: note = mu-conotoxin or tarantula toxin ProTxII amino acid sequence
ERCNGRRGCSRWRDHSRCC

SEQ ID NO: 194 - DNA, 43 bp, synthetic construct
  misc_feature 1..43: note = mu-conotoxin or tarantula toxin ProTxII nucleic acid sequence
  source 1..43: mol_type = other DNA
aggatattgtactaatcggagcaggcagggtgtatgctatacc

SEQ ID NO: 195 - protein, 14 aa, synthetic construct
  REGION 1..14: note = mu-conotoxin or tarantula toxin ProTxII amino acid sequence
GYCTNRSRQGVCYT

SEQ ID NO: 196 - DNA, 61 bp, synthetic construct
  misc_feature 1..61: note = mu-conotoxin or tarantula toxin ProTxII nucleic acid sequence
  source 1..61: mol_type = other DNA
gtattacgattgcaactgcagcagatgggctcgcgaccatagcaggtgctgctattataac

SEQ ID NO: 197 - protein, 20 aa, synthetic construct
  REGION 1..20: note = mu-conotoxin or tarantula toxin ProTxII amino acid sequence
YYDCNCSRWARDHSRCCYYN

SEQ ID NO: 198 - DNA, 76 bp, synthetic construct
  misc_feature 1..76: note = mu-conotoxin or tarantula toxin ProTxII nucleic acid sequence
  source 1..76: mol_type = other DNA
gtattactatgagagatgcaatggcagacgcggctgcagcagatggcgcgatcatagcaggtgctgctattataac

SEQ ID NO: 199 - protein, 25 aa, synthetic construct
  REGION 1..25: note = mu-conotoxin or tarantula toxin ProTxII amino acid sequence
YYYERCNGRRGCSRWRDHSRCCYYN

SEQ ID NO: 200 - DNA, 57 bp, synthetic construct
  misc_feature 1..57: note = mu-conotoxin or tarantula toxin ProTxII nucleic acid sequence
  source 1..57: mol_type = other DNA
gagaggctttgtggcttccctaagagctgcagcaggcaaaagcctcacagatgctgc

SEQ ID NO: 201 - protein, 19 aa, synthetic construct
  REGION 1..19: note = mu-conotoxin or tarantula toxin ProTxII amino acid sequence
ERLCGFPKSCSRQKPHRCC

SEQ ID NO: 202 - DNA, 90 bp, synthetic construct
  misc_feature 1..90: note = mu-conotoxin or tarantula toxin ProTxII nucleic acid sequence
  source 1..90: mol_type = other DNA
tactgccagaagtggatgtggactagcgatagtgagaggaagtgctgtgagggtatggtaagccggctgtggtgtaagaagaagctctgg

SEQ ID NO: 203 - protein, 30 aa, synthetic construct
  REGION 1..30: note = mu-conotoxin or tarantula toxin ProTxII amino acid sequence
YCQKWMWTSDSERKCCEGMVSRLWCKKKLW

SEQ ID NO: 204 - DNA, 38 bp, synthetic construct
  misc_feature 1..38: note = mu-conotoxin or tarantula toxin ProTxII nucleic acid sequence
  source 1..38: mol_type = other DNA
tgcaactgcagcagatggcgcgaccatagcaggtgctg

SEQ ID NO: 205 - protein, 12 aa, synthetic construct
  REGION 1..12: note = mu-conotoxin or tarantula toxin ProTxII amino acid sequence
CNCSRWRDHSRC

SEQ ID NO: 206 - DNA, 66 bp, synthetic construct
  misc_feature 1..66: note = mu-conotoxin or tarantula toxin ProTxII nucleic acid sequence
  source 1..66: mol_type = other DNA
gagagatgctgcaatggcagacgcggctgcagcagcagatggtgccgcgatcatagcaggtgctgc

SEQ ID NO: 207 - protein, 22 aa, synthetic construct
  REGION 1..22: note = mu-conotoxin or tarantula toxin ProTxII amino acid sequence
ERCCNGRRGCSSRWCRDHSRCC

SEQ ID NO: 208 - DNA, 43 bp, synthetic construct
  misc_feature 1..43: note = mu-conotoxin or tarantula toxin ProTxII nucleic acid sequence
  source 1..43: mol_type = other DNA
aggatattgtagtggtagcagcagatggggtagctgctactcc

SEQ ID NO: 209 - protein, 14 aa, synthetic construct
  REGION 1..14: note = mu-conotoxin or tarantula toxin ProTxII amino acid sequence
GYCSGSSRWGSCYS

SEQ ID NO: 210 - DNA, 88 bp, synthetic construct
  misc_feature 1..88: note = mu-conotoxin or tarantula toxin ProTxII nucleic acid sequence
  source 1..88: mol_type = other DNA
gtattatgattacgagagagcttgcaatggcagacgcggctgcagcagatgggctcgcgatcatagcaggtgctgctatcgttatacc

SEQ ID NO: 211 - protein, 29 aa, synthetic construct
  REGION 1..29: note = mu-conotoxin or tarantula toxin ProTxII amino acid sequence
YYDYERACNGRRGCSRWARDHSRCCYRYT

SEQ ID NO: 212 - DNA, 63 bp, synthetic construct
  misc_feature 1..63: note = mu-conotoxin or tarantula toxin ProTxII nucleic acid sequence
  source 1..63: mol_type = other DNA
gagaggcttgcttgtggcttccctaagagctgcagcaggcaagctaagcctcacagatgctgc

SEQ ID NO: 213 - protein, 21 aa, synthetic construct
  REGION 1..21: note = mu-conotoxin or tarantula toxin ProTxII amino acid sequence
ERLACGFPKSCSRQAKPHRCC

SEQ ID NO: 214 - DNA, 90 bp, synthetic construct
  misc_feature 1..90: note = mu-conotoxin or tarantula toxin ProTxII nucleic acid sequence
  source 1..90: mol_type = other DNA
tactgccagaagtggatgtggacttgcgatagtgagaggaagagctgtgagggtatggtatgccggctgtggagtaagaagaagctctgg

SEQ ID NO: 215 - protein, 30 aa, synthetic construct
  REGION 1..30: note = mu-conotoxin or tarantula toxin ProTxII amino acid sequence
YCQKWMWTCDSERKSCEGMVCRLWSKKKLW

SEQ ID NO: 216 - DNA, 41 bp, synthetic construct
  misc_feature 1..41: note = mu-conotoxin or tarantula toxin ProTxII nucleic acid sequence
  source 1..41: mol_type = other DNA
tgcaactgcagcagatgggctcgcgaccatagcaggtgctg

SEQ ID NO: 217 - protein, 13 aa, synthetic construct
  REGION 1..13: note = mu-conotoxin or tarantula toxin ProTxII amino acid sequence
CNCSRWARDHSRC

SEQ ID NO: 218 - DNA, 63 bp, synthetic construct
  misc_feature 1..63: note = mu-conotoxin or tarantula toxin ProTxII nucleic acid sequence
  source 1..63: mol_type = other DNA
gagagagcttgcaatggcagacgcggctgcagcagatgggctcgcgatcatagcaggtgctgc

SEQ ID NO: 219 - protein, 21 aa, synthetic construct
  REGION 1..21: note = mu-conotoxin or tarantula toxin ProTxII amino acid sequence
ERACNGRRGCSRWARDHSRCC

SEQ ID NO: 220 - DNA, 31 bp, synthetic construct
  misc_feature 1..31: note = mu-conotoxin or tarantula toxin ProTxII nucleic acid sequence
  source 1..31: mol_type = other DNA
agcatattgtcggagcaggcagtgctattcc

SEQ ID NO: 221 - protein, 10 aa, synthetic construct
  REGION 1..10: note = mu-conotoxin or tarantula toxin ProTxII amino acid sequence
AYCRSRQCYS

SEQ ID NO: 222 - DNA, 82 bp, synthetic construct
  misc_feature 1..82: note = mu-conotoxin or tarantula toxin ProTxII nucleic acid sequence
  source 1..82: mol_type = other DNA
gtattactatgagaggcttgcttgtggcttccctaagagctgcagcaggcaagctaagcctcacagatgctgctattactac

SEQ ID NO: 223 - protein, 27 aa, synthetic construct
  REGION 1..27: note = mu-conotoxin or tarantula toxin ProTxII amino acid sequence
YYYERLACGFPKSCSRQAKPHRCCYYY

SEQ ID NO: 224 - DNA, 66 bp, synthetic construct
  misc_feature 1..66: note = mu-conotoxin or tarantula toxin ProTxII nucleic acid sequence
  source 1..66: mol_type = other DNA
gagaggctttgctgtggcttccctaagagctgccgcagcaggcaatgcaagcctcacagatgctgc

SEQ ID NO: 225 - protein, 22 aa, synthetic construct
  REGION 1..22: note = mu-conotoxin or tarantula toxin ProTxII amino acid sequence
ERLCCGFPKSCRSRQCKPHRCC

SEQ ID NO: 226 - DNA, 90 bp, synthetic construct
  misc_feature 1..90: note = mu-conotoxin or tarantula toxin ProTxII nucleic acid sequence
  source 1..90: mol_type = other DNA
tactgccagaagtggatgtggacttgcgatagtgagaggaagtgctgtgagggtatggtatgccggctgtggtgtaagaagaagctctgg

SEQ ID NO: 227 - protein, 30 aa, synthetic construct
  REGION 1..30: note = mu-conotoxin or tarantula toxin ProTxII amino acid sequence
YCQKWMWTCDSERKCCEGMVCRLWCKKKLW

SEQ ID NO: 228 - DNA, 48 bp, synthetic construct
  misc_feature 1..48: note = mu-conotoxin or tarantula toxin ProTxII nucleic acid sequence
  source 1..48: mol_type = other DNA
tgctgcaactgcagcagcaaatggtgccgcgaccatagcaggtgctgc

SEQ ID NO: 229 - protein, 16 aa, synthetic construct
  REGION 1..16: note = mu-conotoxin or tarantula toxin ProTxII amino acid sequence
CCNCSSKWCRDHSRCC

SEQ ID NO: 230 - DNA, 77 bp, synthetic construct
  misc_feature 1..77: note = mu-conotoxin or tarantula toxin ProTxII nucleic acid sequence
  source 1..77: mol_type = other DNA
ggtatagtggggagaggctttgtggcttccctaagagctgcagcaggcaaaagcctcacagatgctgcagctactac

SEQ ID NO: 231 - protein, 25 aa, synthetic construct
  REGION 1..25: note = mu-conotoxin or tarantula toxin ProTxII amino acid sequence
YSGERLCGFPKSCSRQKPHRCCSYY

SEQ ID NO: 232 - DNA, 9975 bp, synthetic construct
  misc_feature 1..9975: note = Tx-DH1166
  source 1..9975: mol_type = other DNA
tacgtagccgtttcgatcctcccgaattgactagtgggtaggcctggcggccgctgccatttcattacctctttctccgcacccgacatagataccggtggattcgaattctccccgttgaagctgacctgcccagaggggcctgggcccaccccacacaccggggcggaatgtgtacaggccccggtctctgtgggtgttccgctaactggggctcccagtgctcaccccacaactaaagcgagccccagcctccagagcccccgaaggagatgccgcccacaagcccagcccccatccaggaggccccagagctcagggcgccggggcggattttgtacagccccgagtcactgtggagagaagctgcaatggcagacgcggctgcagcagcagatggagccgcgatcatagcaggtgctgccacagtgagaaaaactgtgtcaaaaaccgtctcctggcccctgctggaggccgcgccagagaggggagcagccgccccgaacctaggtcctgctcagctcacacgacccccagcacccagagcacaacggagtccccattgaatggtgaggacggggaccagggctccagggggtcatggaaggggctggaccccatcctactgctatggtcccagtgctcctggccagaactgaccctaccaccgacaagagtccctcagggaaacgggggtcactggcacctcccagcatcaaccccaggcagcacaggcataaaccccacatccagagccgactccaggagcagagacaccccagtaccctgggggacaccgaccctgatgactccccactggaatccaccccagagtccaccaggaccaaagaccccgcccctgtctctgtccctcactcaggacctgctgcggggcgggccatgagaccagactcgggcttagggaacaccactgtggccccaacctcgaccaggccacaggcccttccttcctgccctgcggcagcacagactttggggtctgtgcagagaggaatcacagaggccccaggctgaggtggtgggggtggaagacccccaggaggtggcccacttcccttcctcccagctggaacccaccatgaccttcttaagataggggtgtcatccgaggcaggtcctccatggagctcccttcaggctcctccccggtcctcactaggcctcagtcccggctgcgggaatgcagccaccacaggcacaccaggcagcccagacccagccagcctgcagtgcccaagcccacattctggagcagagcaggctgtgtctgggagagtctgggctccccaccgcccccccgcacaccccacccacccctgtccaggccctatgcaggagggtcagagccccccatggggtatggacttagggtctcactcacgtggctcccctcctgggtgaaggggtctcatgcccagatccccacagcagagctggtcaaaggtggaggcagtggccccagggccaccctgacctggaccctcaggctcctctagccctggctgccctgctgtccctgggaggcctggactccaccagaccacaggtccagggcaccgcccataggtgctgcccacactcagttcacaggaagaagataagctccagacccccaagactgggacctgccttcctgccaccgcttgtagctccagacctccgtgcctcccccgaccacttacacacgggccagggagctgttccacaaagatcaaccccaaaccgggaccgcctggcactcgggccgctgccacttccctctccatttgttcccagcacctctgtgctccctccctcctccctccttcaggggaacagcctgtgcagcccctccctgcaccccacaccctggggaggcccaaccctgcctccagccctttctcccccgctgctcttcctgcccatccagacaaccctggggtcccatccctgcagcctacaccctggtctccacccagacccctgtctctccctccagacacccctcccaggccaaccctgcacatgcaggccctccccttttctgctgccagagcctcagtttctaccctctgtgcctaccccctgcctcctcctgcccacaactcgagctcttcctctcctggggcccctgagccatggcactgaccgtgcactcccacccccacactgcccatgccctcaccttcctcctggacactctgaccccgctcccctcttggacccagccctggtatttccaggacaaaggctcacccaagtcttccccatgcaggcccttgccctcactgcccggttacacggcagcctcctgtgcacagaagcagggagctcagcccttccacaggcagaaggcactgaaagaaatcggcctccagcaccctgatgcacgtccgcctgtgtctctcactgcccgcacctgcagggaggctcggcactccctgtaaagacgagggatccaggcagcaacatcatgggagaatgcagggctcccagacagcccagccctctcgcaggcctctcctgggaagagacctgcagccaccactgaacagccacggagcccgctggatagtaactgagtcagtgaccgacctggagggcaggggagcagtgaaccggagcccagaccatagggacagagaccagccgctgacatcccgagcccctcactggcggccccagaacaccgcgtggaaacagaacagacccacattcccacctggaacagggcagacactgctgagcccccagcaccagccctgagaaacaccaggcaacggcatcagagggggctcctgagaaagaaaggaggggaggtctccttcaccagcaagtacttcccttgaccaaaaacagggtccacgcaactcccccaggacaaaggaggagccccctgtacagcactgggctcagagtcctctcccacacaccctgagtttcagacaaaaaccccctggaaatcatagtatcagcaggagaactagccagagacagcaagaggggactcagtgactcccgcggggacaggaggattttgtgggggctcgtgtcactgtgaggatattgtagcagcagatggtgctatacccacagtgacacagccccattcaaaaacccctgctgtaaacgcttccacttctggagctgaggggctggggggagcgtctgggaagtagggcctaggggtggccatcaatgcccaaaacgcaccagactcccccccagacatcaccccactggccagtgagcagagtaaacagaaaatgagaagcagctgggaagcttgcacaggccccaaggaaagagctttggcgggtgtgcaagaggggatgcgggcagagcctgagcagggccttttgctgtttctgctttcctgtgcagatagttccataaactggtgttcaagatcgatggctgggagtgagcccaggaggacagtgtgggaagggcacagggaaggagaagcagccgctatcctacactgtcatctttcaagagtttgccctgtgcccacaatgctgcatcatgggatgcttaacagctgatgtagacacagctaaagagagaatcagtgaaatggatttgcagcacagatctgaataaattctccagaatgtggagccacacagaagcaagcacaaggaaagtgcctgatgcaagggcaaagtacagtgtgtaccttcaggctgggcacagacactctgaaaagccttggcaggaactccctgcaacaaagcagagccctgcaggcaatgccagctccagagccctccctgagagcctcatgggcaaagatgtgcacaacaggtgtttctcatagccccaaactgagaatgaagcaaacagccatctgaaggaaaacaggcaaataaacgatggcaggttcatgaaatgcaaacccagacagccagaaggacaacagtgagggttacaggtgactctgtggttgagttcatgacaatgctgagtaattggagtaacaaaggaaagtccaaaaaatactttcaatgtgatttcttctaaataaaatttacagccggcaaaatgaactatcttcttaagggataaactttccactaggaaaactataaggaaaatcaagaaaaggatgatcacataaacacagtggtcgttacttctactggggaaggaagagggtatgaactgagacacacagggttggcaagtctcctaacaagaacagaacaaatacattacagtaccttgaaaacagcagttaaaattctaaattgcaagaagaggaaaatgcacacagctgtgtttagaaaattctcagtccagcactgttcataatagcaaagacattaacccaggttggataaataaacgatgacacaggcaattgcacaatgatacagacatacattcagtatatgagacattgatgatgtatccccaaagaaatgactttaaagagaaaaggcctgatatgtggtggcactcacctccctgggcatccccggacaggctgcaggcacactgtgtggcagggcaggctggtacctgctggcagctcctggggcctgatgtggagcaggcacagagccgtatccccccgaggacatatacccccaaggacggcacagttggtacattccggagacaagcaactcagccacactcccaggccagagcccgagagggacgcccatgcacagggaggcagagcccagctcctccacagccagcagcacccgtgcaggggccgccatctggcaggcacagagcatgggctgggaggaggggcagggacaccaggcagggttggcaccaactgaaaattacagaagtctcatacatctacctcagccttgcctgacctgggcctcacctgacctggacctcacctggcctggacctcacctggcctagacctcacctctgggcttcacctgagctcggcctcacctgacttggaccttgcctgtcctgagctcacatgatctgggcctcacctgacctgggtttcacctgacctgggcttcacctgacctgggcctcatctgacctgggcctcactggcctggacctcacctggcctgggcttcacctggcctcaggcctcatctgcacctgctccaggtcttgctggaacctcagtagcactgaggctgcaggggctcatccagggttgcagaatgactctagaacctcccacatctcagctttctgggtggaggcacctggtggcccagggaatataaaaagcctgaatgatgcctgcgtgatttgggggcaatttataaacccaaaaggacatggccatgcagcgggtagggacaatacagacagatatcagcctgaaatggagcctcagggcacaggtgggcacggacactgtccacctaagccaggggcagacccgagtgtccccgcagtagacctgagagcgctgggcccacagcctcccctcggtgccctgctacctcctcaggtcagccctggacatcccgggtttccccaggcctggcggtaggattttgttgaggtctgtgtcactgtggtattacgattgcaactgcagcagatggcgcgaccatagcaggtgctgctattatacccacagtgtcacagagtccatcaaaaacccatccctgggaaccttctgccacagccctccctgtggggcaccgccgcgtgccatgttaggattttgactgaggacacagcaccatgggtatggtggctaccgcagcagtgcagcccgtgacccaaacacacagggcagcaggcacaacagacaagcccacaagtgaccaccctgagctcctgcctgccagccctggagaccatgaaacagatggccaggattatcccataggtcagccagacctcagtccaacaggtctgcatcgctgctgccctccaataccagtccggatggggacagggctggcccacattaccatttgctgccatccggccaacagtcccagaagcccctccctcaaggctgggccacatgtgtggaccctgagagccccccatgtctgagtaggggcaccaggaaggtggggctggccctgtgcactgtccctgcccctgtggtccctggcctgcctggccctgacacctgggcctctcctgggtcatttccaagacagaagacattcccaggacagctggagctgggagtccatcatcctgcctggccgtcctgagtcctgcgcctttccaaacctcacccgggaagccaacagaggaatcacctcccacaggcagagacaaagaccttccagaaatctctgtctctctccccagtgggcaccctcttccagggcagtcctcagtgatatcacagtgggaacccacatctggatcgggactgcccccagaacacaagatggcccacagggacagccccacagcccagcccttcccagacccctaaaaggcgtcccaccccctgcatctgccccagggctcaaactccaggaggactgactcctgcacaccctcctgccagacatcacctcagcccctcctggaagggacaggagcgcgcaagggtgagtcagaccctcctgccctcgatggcaggcggagaagattcagaaaggtctgagatccccaggacgcagcaccactgtcaatgggggccccagacgcctggaccagggcctgcgtgggaaaggcctctgggcacactcagggggattttgtgaagggtcctcccactgtggagaggcttagctgtggcttccctaagagctgccgcagcaggcaaagcaagcctcacagatgctgccacagtgatgaacccagcatcaaaaaccgaccggactcccaaggtttatgcacacttctccgctcagagctctccaggatcagaagagccgggcccaagggtttctgcccagaccctcggcctctagggacatcttggccatgacagcccatgggctggtgccccacacatcgtctgccttcaaacaagggcttcagagggctctgaggtgacctcactgatgaccacaggtgccctggccccttccccaccagctgcaccagaccccgtcatgacagatgccccgattccaacagccaattcctggggccaggaatcgctgtagacaccagcctccttccaacacctcctgccaattgcctggattcccatcccggttggaatcaagaggacagcatcccccaggctcccaacaggcaggactcccacaccctcctctgagaggccgctgtgttccgtagggccaggctgcagacagtccccctcacctgccactagacaaatgcctgctgtagatgtccccacctggaaaataccactcatggagcccccagccccaggtacagctgtagagagagtctctgaggcccctaagaagtagccatgcccagttctgccgggaccctcggccaggctgacaggagtggacgctggagctgggcccatactgggccacataggagctcaccagtgagggcaggagagcacatgccggggagcacccagcctcctgctgaccagaggcccgtcccagagcccaggaggctgcagaggcctctccagggggacactgtgcatgtctggtccctgagcagccccccacgtccccagtcctgggggcccctggcacagctgtctggaccctctctattccctgggaagctcctcctgacagccccgcctccagttccaggtgtggattttgtcagggggtgtcacactgtgtacagccagaagtggatgtggacttgcgatagtgagaggaagtgcagtgagggtatggtatgccggctgtggtgtaagaagaagctctggcacagtggtgctgcccatatcaaaaaccaggccaagtagacaggcccctgctgtgcagccccaggcctccagctcacctgcttctcctggggctctcaaggctgctgttttctgcactctcccctctgtggggagggttccctcagtgggagatctgttctcaacatcccacggcctcattcctgcaaggaaggccaatggatgggcaacctcacatgccgcggctaagatagggtgggcagcctggcggggacaggacatcctgctggggtatctgtcactgtgcctagtggggcactggctcccaaacaacgcagtccttgccaaaatccccacggcctcccccgctaggggctggcctgatctcctgcagtcctaggaggctgctgacctccagaatggctccgtccccagttccagggcgagagcagatcccaggccggctgcagactgggaggccaccccctccttcccagggttcactgcaggtgaccagggcaggaaatggcctgaacacagggataaccgggccatcccccaacagagtccaccccctcctgctctgtaccccgcaccccccaggccagcccatgacatccgacaaccccacaccagagtcactgcccggtgctgccctagggaggacccctcagcccccaccctgtctagaggactggggaggacaggacacgccctctccttatggttcccccacctggctctggctgggacccttggggtgtggacagaaaggacgcttgcctgattggcccccaggagcccagaacttctctccagggaccccagcccgagcacccccttacccaggacccagccctgcccctcctcccctctgctctcctctcatcaccccatgggaatccagaatccccaggaagccatcaggaagggctgagggaggaagtggggccactgcaccaccaggcaggaggctctgtctttgtgaacccagggaggtgccagcctcctagagggtatggtccaccctgcctatggctcccacagtggcaggctgcagggaaggaccagggacggtgtgggggagggctcagggccccgcgggtgctccatcttggatgagcctatctctctcacccacggactcgcccacctcctcttcaccctggccacacgtcgtccacaccatcctaagtcccacctacaccagagccggcacagccagtgcagacagaggctggggtgcaggggggccgactgggcagcttcggggagggaggaatggaggaaggggagttcagtgaagaggcccccctcccctgggtccaggatcctcctctgggacccccggatcccatcccctccaggctctgggaggagaagcaggatgggagaatctgtgcgggaccctctcacagtggaatacctccacagcggctcaggccagatacaaaagcccctcagtgagccctccactgcagtgctgggcctgggggcagccgctcccacacaggatgaacccagcaccccgaggatgtcctgccagggggagctcagagccatgaaggagcaggatatgggacccccgatacaggcacagacctcagctccattcaggactgccacgtcctgccctgggaggaacccctttctctagtccctgcaggccaggaggcagctgactcctgacttggacgcctattccagacaccagacagaggggcaggccccccagaaccagggatgaggacgccccgtcaaggccagaaaagaccaagttgcgctgagcccagcaagggaaggtccccaaacaaaccaggaggattttgtaggtgtctgtgtcactgtgagctgcaactgcagcagcaaatggagccgcgaccatagcaggtgctgccacagtgacactcgccaggtcaaaaaccccatcccaagtcagcggaatgcagagagagcagggaggacatgtttaggatctgaggccgcacctgacacccaggccagcagacgtctcctgtccacggcaccctgccatgtcctgcatttctggaagaacaagggcaggctgaagggggtccaggaccaggagatgggtccgctctacccagagaaggagccaggcaggacacaagcccccacgcgtgggctcgtagtttgacgtgcgtgaagtgtgggtaagaaagtacgta

SEQ ID NO: 233 - DNA, 9714 bp, synthetic construct
  misc_feature 1..9714: note = TxDH17613
  source 1..9714: mol_type = other DNA
gcggccgctgccatttcattacctctttctccgcacccgacatagattacgtaacgcgtgggctcgtagtttgacgtgcgtgaagtgtgggtaagaaagtccccattgaggctgacctgcccagagggtcctgggcccacccaacacaccggggcggaatgtgtgcaggcctcggtctctgtgggtgttccgctagctggggctcacagtgctcaccccacacctaaaacgagccacagcctccggagcccctgaaggagaccccgcccacaagcccagcccccacccaggaggccccagagcacagggcgccccgtcggattttgtacagccccgagtcactgtggagagatgcaatggcagacgcggctgcagcagatggcgcgatcatagcaggtgctgccacagtgagaaaagcttcgtcaaaaaccgtctcctggccacagtcggaggccccgccagagaggggagcagccaccccaaacccatgttctgccggctcccatgaccccgtgcacctggagccccacggtgtccccactggatgggaggacaagggccgggggctccggcgggtcggggcaggggcttgatggcttccttctgccgtggccccattgcccctggctggagttgacccttctgacaagtgtcctcagagagtcagggatcagtggcacctcccaacatcaaccccacgcagcccaggcacaaaccccacatccagggccaactccaggaacagagacaccccaataccctgggggaccccgaccctgatgactcccgtcccatctctgtccctcacttggggcctgctgcggggcgagcacttgggagcaaactcaggcttaggggacaccactgtgggcctgacctcgagcaggccacagacccttccctcctgccctggtgcagcacagactttggggtctgggcagggaggaacttctggcaggtcaccaagcacagagcccccaggctgaggtggccccagggggaaccccagcaggtggcccactacccttcctcccagctggaccccatgtcttccccaagataggggtgccatccaaggcaggtcctccatggagcccccttcaggctcctctccagaccccactgggcctcagtccccactctaggaatgcagccaccacgggcacaccaggcagcccaggcccagccaccctgcagtgcccaagcccacaccctggaggagagcagggtgcgtctgggaggggctgggctccccacccccacccccacctgcacaccccacccacccttgcccgggccccctgcaggagggtcagagcccccatgggatatggacttagggtctcactcacgcacctcccctcctgggagaaggggtctcatgcccagatccccccagcagcgctggtcacaggtagaggcagtggccccagggccaccctgacctggcccctcaggctcctctagccctggctgccctgctgtccctgggaggcctgggctccaccagaccacaggtctagggcaccgcccacactggggccgcccacacacagctcacaggaagaagataagctccagacccccaggcccgggacctgccttgctgctacgacttcctgccccagacctcgttgccctcccccgtccacttacacacaggccaggaagctgttcccacacagaccaaccccagacggggaccacctggcactcaggtcactgccatttccttctccattcacttccaatgcctctgtgcttcctccctcctccttccttcgggggagcaccctgtgcagctcctccctgcagtccacaccctggggagacccgaccctgcagcccacaccctggggagacctgaccctcctccagccctttctcccccgctgctcttgccacccaccaagacagccctggggtcctgtccctacagcccccacccagttctctacctagacccgtcttcctccctctaaacacctctcccaggccaaccctacacctgcaggccctcccctccactgccaaagaccctcagtttctcctgcctgtgcccacccccgtgctcctcctgcccacagctcgagctcttcctctcctagggcccctgagggatggcattgaccgtgccctcgcacccacacactgcccatgccctcacattcctcctggccactccagccccactcccctctcaggcctggctctggtatttctgggacaaagccttacccaagtctttcccatgcaggcctgggcccttaccctcactgcccggttacagggcagcctcctgtgcacagaagcagggagctcagcccttccacaggcagaaggcactgaaagaaatcggcctccagcgccttgacacacgtctgcctgtgtctctcactgcccgcacctgcagggaggctcggcactccctctaaagacgagggatccaggcagcagcatcacaggagaatgcagggctaccagacatcccagtcctctcacaggcctctcctgggaagagacctgaagacgcccagtcaacggagtctaacaccaaacctccctggaggccgatgggtagtaacggagtcattgccagacctggaggcaggggagcagtgagcccgagcccacaccatagggccagaggacagccactgacatcccaagccactcactggtggtcccacaacaccccatggaaagaggacagacccacagtcccacctggaccagggcagagactgctgagacccagcaccagaaccaaccaagaaacaccaggcaacagcatcagagggggctctggcagaacagaggaggggaggtctccttcaccagcaggcgcttcccttgaccgaagacaggatccatgcaactcccccaggacaaaggaggagccccttgttcagcactgggctcagagtcctctccaagacacccagagtttcagacaaaaaccccctggaatgcacagtctcagcaggagagccagccagagccagcaagatggggctcagtgacacccgcagggacaggaggattttgtgggggctcgtgtcactgtgaggatattgtactaatcggagcaggcagggtgtatgctatacccacagtgacacagccccattcaaaaacccctactgcaaacgcattccacttctggggctgaggggctgggggagcgtctgggaaatagggctcaggggtgtccatcaatgcccaaaacgcaccagactcccctccatacatcacacccaccagccagcgagcagagtaaacagaaaatgagaagcaagctggggaagcttgcacaggccccaaggaaagagctttggcgggtgtgtaagaggggatgcgggcagagcctgagcagggccttttgctgtttctgctttcctgtgcagagagttccataaactggtgttcgagatcaatggctgggagtgagcccaggaggacagcgtgggaagagcacagggaaggaggagcagccgctatcctacactgtcatctttcgaaagtttgccttgtgcccacactgctgcatcatgggatgcttaacagctgatgtagacacagctaaagagagaatcagtgagatggatttgcagcacagatctgaataaattctccagaatgtggagcagcacagaagcaagcacacagaaagtgcctgatgcaaggacaaagttcagtgggcaccttcaggcattgctgctgggcacagacactctgaaaagccctggcaggaactccctgtgacaaagcagaaccctcaggcaatgccagccccagagccctccctgagagcctcatgggcaaagatgtgcacaacaggtgtttctcatagccccaaactgagagcaaagcaaacgtccatctgaaggagaacaggcaaataaacgatggcaggttcatgaaatgcaaacccagacagccacaagcacaaaagtacagggttataagcgactctggttgagttcatgacaatgctgagtaattggagtaacaaagtaaactccaaaaaatactttcaatgtgatttcttctaaataaaatttacaccctgcaaaatgaactgtcttcttaagggatacatttcccagttagaaaaccataaagaaaaccaagaaaaggatgatcacataaacacagtggtggttacttctgctggggaaggaagagggtatgaactgagatacacagggtgggcaagtctcctaacaagaacagaacgaatacattacagtaccttgaaaacagcagttaaacttctaaattgcaagaagaggaaaatgcacacagttgtgtttagaaaattctcagtccagcactgttcataatagcaaagacattaacccaggtcggataaataagcgatgacacaggcaattgcacaatgatacagacatatatttagtatatgagacatcgatgatgtatccccaaataaacgactttaaagagataaagggctgatgtgtggtggcattcacctccctgggatccccggacaggttgcaggctcactgtgcagcagggcaggcgggtacctgctggcagttcctggggcctgatgtggagcaagcgcagggccatatatcccggaggacggcacagtcagtgaattccagagagaagcaactcagccacactccccaggcagagcccgagagggacgcccacgcacagggaggcagagcccagcacctccgcagccagcaccacctgcgcacgggccaccaccttgcaggcacagagtgggtgctgagaggaggggcagggacaccaggcagggtgagcacccagagaaaactgcagacgcctcacacatccacctcagcctcccctgacctggacctcactggcctgggcctcacttaacctgggcttcacctgaccttggcctcacctgacttggacctcgcctgtcccaagctttacctgacctgggcctcaactcacctgaacgtctcctgacctgggtttaacctgtcctggaactcacctggccttggcttcccctgacctggacctcatctggcctgggcttcacctggcctgggcctcacctgacctggacctcatctggcctggacctcacctggcctggacttcacctggcctgggcttcacctgacctggacctcacctggcctcgggcctcacctgcacctgctccaggtcttgctggagcctgagtagcactgagggtgcagaagctcatccagggttggggaatgactctagaagtctcccacatctgacctttctgggtggaggcagctggtggccctgggaatataaaaatctccagaatgatgactctgtgatttgtgggcaacttatgaacccgaaaggacatggccatggggtgggtagggacatagggacagatgccagcctgaggtggagcctcaggacacaggtgggcacggacactatccacataagcgagggatagacccgagtgtccccacagcagacctgagagcgctgggcccacagcctcccctcagagccctgctgcctcctccggtcagccctggacatcccaggtttccccaggcctggcggtaggattttgttgaggtctgtgtcactgtggtattacgattgcaactgcagcagatgggctcgcgaccatagcaggtgctgctattataaccacagtgtcacagagtccatcaaaaacccatgcctggaagcttcccgccacagccctccccatggggccctgctgcctcctcaggtcagccccggacatcccgggtttccccaggctgggcggtaggattttgttgaggtctgtgtcactgtggtattactatgagagatgcaatggcagacgcggctgcagcagatggcgcgatcatagcaggtgctgctattataaccacagtgtcacagagtccatcaaaaacccatccctgggagcctcccgccacagccctccctgcaggggaccggtacgtgccatgttaggattttgatcgaggagacagcaccatgggtatggtggctaccacagcagtgcagcctgtgacccaaacccgcagggcagcaggcacgatggacaggcccgtgactgaccacgctgggctccagcctgccagccctggagatcatgaaacagatggccaaggtcaccctacaggtcatccagatctggctccgaggggtctgcatcgctgctgccctcccaacgccagtccaaatgggacagggacggcctcacagcaccatctgctgccatcaggccagcgatcccagaagcccctccctcaaggctgggcacatgtgtggacactgagagccctcatatctgagtaggggcaccaggagggaggggctggccctgtgcactgtccctgcccctgtggtccctggcctgcctggccctgacacctgagcctctcctgggtcatttccaagacagaagacattcctggggacagccggagctgggcgtcgctcatcctgcccggccgtcctgagtcctgctcatttccagacctcaccggggaagccaacagaggactcgcctcccacattcagagacaaagaaccttccagaaatccctgcctctctccccagtggacaccctcttccaggacagtcctcagtggcatcacagcggcctgagatccccaggacgcagcaccgctgtcaataggggccccaaatgcctggaccagggcctgcgtgggaaaggcctctggccacactcggggattttgtgaagggccctcccactgtggagaggctttgtggcttccctaagagctgcagcaggcaaaagcctcacagatgctgccacagtgatgaacccagtgtcaaaaaccggctggaaacccaggggctgtgtgcacgcctcagcttggagctctccaggagcacaagagccgggcccaaggatttgtgcccagaccctcagcctctagggacacctgggtcatctcagcctgggctggtgccctgcacaccatcttcctccaaataggggcttcagagggctctgaggtgacctcactcatgaccacaggtgacctggcccttccctgccagctataccagaccctgtcttgacagatgccccgattccaacagccaattcctgggaccctgaatagctgtagacaccagcctcattccagtacctcctgccaattgcctggattcccatcctggctggaatcaagaaggcagcatccgccaggctcccaacaggcaggactcccgcacaccctcctctgagaggccgctgtgttccgcagggccaggccctggacagttcccctcacctgccactagagaaacacctgccattgtcgtccccacctggaaaagaccactcgtggagcccccagccccaggtacagctgtagagacagtcctcgaggcccctaagaaggagccatgcccagttctgccgggaccctcggccaggccgacaggagtggacgctggagctgggcccacactgggccacataggagctcaccagtgagggcaggagagcacatgccggggagcacccagcctcctgctgaccagaggcccgtcccagagcccaggaggctgcagaggcctctccagggagacactgtgcatgtctggtacctaagcagccccccacgtccccagtcctgggggcccctggctcagctgtctgggccctccctgctccctgggaagctcctcctgacagccccgcctccagttccaggtgtggattttgtcaggcgatgtcacactgtgtactgccagaagtggatgtggactagcgatagtgagaggaagtgctgtgagggtatggtaagccggctgtggtgtaagaagaagctctggcacagtggtgccgcccatatcaaaaaccaggccaagtagacaggcccctgctgcgcagccccaggcatccacttcacctgcttctcctggggctctcaaggctgctgtctgtcctctggccctctgtggggagggttccctcagtgggaggtctgtgctccagggcagggatgattgagatagaaatcaaaggctggcagggaaaggcagcttcccgccctgagaggtgcaggcagcaccacggagccacggagtcacagagccacggagcccccattgtgggcatttgagagtgctgtgcccccggcaggcccagccctgatggggaagcctgtcccatcccacagcccgggtcccacgggcagcgggcacagaagctgccaggttgtcctctatgatcctcatccctccagcagcatcccctccacagtggggaaactgaggcttggagcaccacccggccccctggaaatgaggctgtgagcccagacagtgggcccagagcactgtgagtaccccggcagtacctggctgcagggatcagccagagatgccaaaccctgagtgaccagcctacaggaggatccggccccacccaggccactcgattaatgctcaaccccctgccctggagacctcttccagtaccaccagcagctcagcttctcagggcctcatccctgcaaggaaggtcaagggctgggcctgccagaaacacagcaccctccctagccctggctaagacagggtgggcagacggctgtggacgggacatattgctggggcatttctcactgtcacttctgggtggtagctctgacaaaaacgcagaccctgccaaaatccccactgcctcccgctaggggctggcctggaatcctgctgtcctaggaggctgctgacctccaggatggctccgtccccagttccagggcgagagcagatcccaggcaggctgtaggctgggaggccacccctgcccttgccggggttgaatgcaggtgcccaaggcaggaaatggcatgagcacagggatgaccgggacatgccccaccagagtgcgccccttcctgctctgcaccctgcaccccccaggccagcccacgacgtccaacaactgggcctgggtggcagccccacccagacaggacagacccagcaccctgaggaggtcctgccagggggagctaagagccatgaaggagcaagatatggggcccccgatacaggcacagatgtcagctccatccaggaccacccagcccacaccctgagaggaacgtctgtctccagcctctgcaggtcgggaggcagctgacccctgacttggacccctattccagacaccagacagaggcgcaggccccccagaaccagggttgagggacgccccgtcaaagccagacaaaaccaaggggtgttgagcccagcaagggaaggcccccaaacagaccaggaggattttgtaggtgtctgtgtcactgtgtgcaactgcagcagatggcgcgaccatagcaggtgctgccacagtgacactcacccagtcaaaaaccccattccaagtcagcggaagcagagagagcagggaggacacgtttaggatctgagactgcacctgacacccaggccagcagacgtctcccctccagggcaccccaccctgtcctgcatttctgcaagatcaggggcggcctgagggggggtctagggtgaggagatgggtcccctgtacaccaaggaggagttaggcaggtcccgagcactcttaattaaacgacgcctcgaatggaactactacaacgaatggttgctctacgtaatgcattcgctaccttaggaccgttatagttaggcgcgcc

SEQ ID NO: 234 - DNA, 9797 bp, synthetic construct
  misc_feature 1..9797: note = TxDH114619
  source 1..9797: mol_type = other DNA
tacgtattaattaaacgacgcctcgaatggaactactacaacgaatggttgctctccccattgaggctgacctgcccagagagtcctgggcccaccccacacaccggggcggaatgtgtgcaggcctcggtctctgtgggtgttccgctagctggggctcacagtgctcaccccacacctaaaatgagccacagcctccggagcccccgcaggagaccccgcccacaagcccagcccccacccaggaggccccagagctcagggcgccccgtcggattttgtacagccccgagtcactgtggagagatgctgcaatggcagacgcggctgcagcagcagatggtgccgcgatcatagcaggtgctgccacagtgagaatagctacgtcaaaaaccgtccagtggccactgccggaggccccgccagagagggcagcagccactctgatcccatgtcctgccggctcccatgacccccagcacgcggagccccacagtgtccccactggatgggaggacaagagctggggattccggcgggtcggggcaggggcttgatcgcatccttctgccgtggctccagtgcccctggctggagttgacccttctgacaagtgtcctcagagagacaggcatcaccggcgcctcccaacatcaaccccaggcagcacaggcacaaaccccacatccagagccaactccaggagcagagacaccccaataccctgggggaccccgaccctgatgacttcccactggaattcgccgtagagtccaccaggaccaaagaccctgcctctgcctctgtccctcactcaggacctgctgccgggcgaggccttgggagcagacttgggcttaggggacaccagtgtgaccccgaccttgaccaggacgcagacctttccttcctttcctggggcagcacagactttggggtctgggccaggaggaacttctggcaggtcgccaagcacagaggccacaggctgaggtggccctggaaagacctccaggaggtggccactccccttcctcccagctggaccccatgtcctccccaagataagggtgccatccaaggcaggtgctccttggagccccattcagactcctccctggaccccactgggcctcagtcccagctctggggatgaagccaccacaagcacaccaggcagcccaggcccagccaccctgcagtgcccaagcacacactctggagcagagcagggtgcctctgggaggggctgagctccccaccccacccccacctgcacaccccacccacccctgcccagcggctctgcaggagggtcagagccccacatggggtatggacttagggtctcactcacgtggctcccatcatgagtgaaggggcctcaagcccaggttcccacagcagcgcctgtcgcaagtggaggcagaggcccgagggccaccctgacctggtccctgaggttcctgcagcccaggctgccctgctgtccctgggaggcctgggctccaccagaccacaggtccagggcaccgggtgcaggagccacccacacacagctcacaggaagaagataagctccagacccccagggccagaacctgccttcctgctactgcttcctgccccagacctgggcgccctcccccgtccacttacacacaggccaggaagctgttcccacacagaacaaccccaaaccaggaccgcctggcactcaggtggctgccatttccttctccatttgctcccagcgcctctgtcctccctggttcctccttcgggggaacagcctgtgcagccagtccctgcagcccacaccctggggagacccaaccctgcctggggcccttccaaccctgctgctcttactgcccacccagaaaactctggggtcctgtccctgcagtccctaccctggtctccacccagacccctgtgtatcactccagacacccctcccaggcaaaccctgcacctgcaggccctgtcctcttctgtcgctagagcctcagtttctcccccctgtgcccacaccctacctcctcctgcccacaactctaactcttcttctcctggagcccctgagccatggcattgaccctgccctcccaccacccacagcccatgccctcaccttcctcctggccactccgaccccgccccctctcaggccaagccctggtatttccaggacaaaggctcacccaagtctttcccaggcaggcctgggctcttgccctcacttcccggttacacgggagcctcctgtgcacagaagcagggagctcagcccttccacaggcagaaggcactgaaagaaatcggcctccagcaccttgacacacgtccgcccgtgtctctcactgcccgcacctgcagggaggctccgcactccctctaaagacaagggatccaggcagcagcatcacgggagaatgcagggctcccagacatcccagtcctctcacaggcctctcctgggaagagacctgcagccaccaccaaacagccacagaggctgctggatagtaactgagtcaatgaccgacctggagggcaggggagcagtgagccggagcccataccatagggacagagaccagccgctgacatcccgagctcctcaatggtggccccataacacacctaggaaacataacacacccacagccccacctggaacagggcagagactgctgagcccccagcaccagccccaagaaacaccaggcaacagtatcagagggggctcccgagaaagagaggaggggagatctccttcaccatcaaatgcttcccttgaccaaaaacagggtccacgcaactcccccaggacaaaggaggagccccctatacagcactgggctcagagtcctctctgagacaccctgagtttcagacaacaacccgctggaatgcacagtctcagcaggagaacagaccaaagccagcaaaagggacctcggtgacaccagtagggacaggaggattttgtgggggctcgtgtcactgtgaggatattgtagtggtagcagcagatggggtagctgctactcccacagtgacacagacccattcaaaaacccctactgcaaacacacccactcctggggctgaggggctgggggagcgtctgggaagtagggtccaggggtgtctatcaatgtccaaaatgcaccagactccccgccaaacaccaccccaccagccagcgagcagggtaaacagaaaatgagaggctctgggaagcttgcacaggccccaaggaaagagctttggcgggtgtgcaagaggggatgcaggcagagcctgagcagggccttttgctgtttctgctttcctgtgcagagagttccataaactggtgttcaagatcagtggctgggaatgagcccaggagggcagtctgtgggaagagcacagggaaggaggagcagccgctatcctacactgtcatctttcaaaagtttgccttgtgaccacactattgcatcatgggatgcttaagagctgatgtagacacagctaaagagagaatcagtgagatgaatttgcagcatagatctgaataaactctccagaatgtggagcagtacagaagcaaacacacagaaagtgcctgatgcaaggacaaagttcagtgggcaccttcaggcattgctgctgggcacagacactctgaaaagccttggcaggatctccctgcgacaaagcagaaccctcaggcaatgccagccccagagccctccctgagagcgtcatggggaaagatgtgcagaacagctgattatcatagactcaaactgagaacagagcaaacgtccatctgaagaacagtcaaataagcaatggtaggttcatgcaatgcaaacccagacagccaggggacaacagtagagggctacaggcggctttgcggttgagttcatgacaatgctgagtaattggagtaacagaggaaagcccaaaaaatacttttaatgtgatttcttctaaataaaatttacaccaggcaaaatgaactgtcttcttaagggataaactttcccctggaaaaactacaaggaaaattaagaaaacgatgatcacataaacacagttgtggttacttctactggggaaggaagagggtatgagctgagacacacagagtcggcaagtctccaagcaagcacagaacgaatacattacagtaccttgaatacagcagttaaacttctaaatcgcaagaacaggaaaatgcacacagctgtgtttagaaaattctcagtccagcactattcataatagcaaagacattaacccaggttggataaataaatgatgacacaggcaattgcacaatgatacagacatacatttagtacatgagacatcgatgatgtatccccaaagaaatgactttaaagagaaaaggcctgatgtgtggtggcactcacctccctgggatccccggacaggttgcaggcacactgtgtggcagggcaggctggtacatgctggcagctcctggggcctgatgtggagcaagcgcagggctgtatacccccaaggatggcacagtcagtgaattccagagagaagcagctcagccacactgcccaggcagagcccgagagggacgcccacgtacagggaggcagagcccagctcctccacagccaccaccacctgtgcacgggccaccaccttgcaggcacagagtgggtgctgagaggaggggcagggacaccaggcagggtgagcacccagagaaaactgcagaagcctcacacatccacctcagcctcccctgacctggacctcacctggtctggacctcacctggcctgggcctcacctgacctggacctcacctggcctgggcttcacctgacctggacctcacctggcctccggcctcacctgcacctgctccaggtcttgctggaacctgagtagcactgaggctgcagaagctcatccagggttggggaatgactctggaactctcccacatctgacctttctgggtggaggcatctggtggccctgggaatataaaaagccccagaatggtgcctgcgtgatttgggggcaatttatgaacccgaaaggacatggccatggggtgggtagggacatagggacagatgccagcctgaggtggagcctcaggacacagttggacgcggacactatccacataagcgagggacagacccgagtgttcctgcagtagacctgagagcgctgggcccacagcctcccctcggtgccctgctgcctcctcaggtcagccctggacatcccgggtttccccaggccagatggtaggattttgttgaggtctgtgtcactgtggtattatgattacgagagagcttgcaatggcagacgcggctgcagcagatgggctcgcgatcatagcaggtgctgctatcgttatacccacagtgtcacacggtccatcaaaaacccatgccacagccctccccgcaggggaccgccgcgtgccatgttacgattttgatcgaggacacagcgccatgggtatggtggctaccacagcagtgcagcccatgacccaaacacacagggcagcaggcacaatggacaggcctgtgagtgaccatgctgggctccagcccgccagccccggagaccatgaaacagatggccaaggtcaccccacagttcagccagacatggctccgtggggtctgcatcgctgctgccctctaacaccagcccagatggggacaaggccaaccccacattaccatctcctgctgtccacccagtggtcccagaagcccctccctcatggctgagccacatgtgtgaaccctgagagcaccccatgtcagagtaggggcagcagaagggcggggctggccctgtgcactgtccctgcacccatggtccctcgcctgcctggccctgacacctgagcctcttctgagtcatttctaagatagaagacattcccggggacagccggagctgggcgtcgctcatcccgcccggccgtcctgagtcctgcttgtttccagacctcaccagggaagccaacagaggactcacctcacacagtcagagacaaagaaccttccagaaatccctgtctcactccccagtgggcaccttcttccaggacattcctcggtcgcatcacagcaggcacccacatctggatcaggacggcccccagaacacaagatggcccatggggacagccccacaacccaggccttcccagacccctaaaaggcgtcccaccccctgcacctgccccagggctaaaaatccaggaggcttgactcccgcataccctccagccagacatcacctcagccccctcctggaggggacaggagcccgggagggtgagtcagacccacctgccctcgatggcaggcggggaagattcagaaaggcctgagatccccaggacgcagcaccactgtcaatgggggccccagacgcctggaccagggcctgcgtgggaaaggccgctgggcacactcagggggattttgtgaaggcccctcccactgtggagaggcttgcttgtggcttccctaagagctgcagcaggcaagctaagcctcacagatgctgccacagtgatgaaactagcatcaaaaaccggccggacacccagggaccatgcacacttctcagcttggagctctccaggaccagaagagtcaggtctgagggtttgtagccagaccctcggcctctagggacaccctggccatcacagcggatgggctggtgccccacatgccatctgctccaaacaggggcttcagagggctctgaggtgacttcactcatgaccacaggtgccctggccccttccccgccagctacaccgaaccctgtcccaacagctgccccagttccaacagccaattcctggggcccagaattgctgtagacaccagcctcgttccagcacctcctgccaattgcctggattcacatcctggctggaatcaagagggcagcatccgccaggctcccaacaggcaggactcccgcacaccctcctctgagaggccgctgtgttccgcagggccaggccctggacagttcccctcacctgccactagagaaacacctgccattgtcgtccccacctggaaaagaccactcgtggagcccccagccccaggtacagctgtagagagactccccgagggatctaagaaggagccatgcgcagttctgccgggaccctcggccaggccgacaggagtggacactggagctgggcccacactgggccacataggagctcaccagtgagggcaggagagcacatgccggggagcacccagcctcctgctgaccagaggcccgtcccagagcccaggaggctgcagaggcctctccagggggacactgtgcatgtctggtccctgagcagccccccacgtccccagtcctgggggcccctggcacagctgtctggaccctccctgttccctgggaagctcctcctgacagccccgcctccagttccaggtgtggattttgtcagggggtgtcacactgtgtactgccagaagtggatgtggacttgcgatagtgagaggaagagctgtgagggtatggtatgccggctgtggagtaagaagaagctctggcacagtggtgctgcccatatcaaaaaccaggccaagtagacaggcccctgctgtgcagccccaggcctccacttcacctgcttctcctggggctctcaaggtcactgttgtctgtactctgccctctgtggggagggttccctcagtgggaggtctgttctcaacatcccagggcctcatgtctgcacggaaggccaatggatgggcaacctcacatgccgcggctaagatagggtgggcagcctggcgggggacagtacatactgctggggtgtctgtcactgtgcctagtggggcactggctcccaaacaacgcagtcctcgccaaaatccccacagcctcccctgctaggggctggcctgatctcctgcagtcctaggaggctgctgacctccagaatgtctccgtccccagttccagggcgagagcagatcccaggccggctgcagactgggaggccaccccctccttcccagggttcactggaggtgaccaaggtaggaaatggccttaacacagggatgactgcgccatcccccaacagagtcagccccctcctgctctgtaccccgcaccccccaggccagtccacgaaaaccagggccccacatcagagtcactgcctggcccggccctggggcggacccctcagcccccaccctgtctagaggacttggggggacaggacacaggccctctccttatggttcccccacctgcctccggccgggacccttggggtgtggacagaaaggacacctgcctaattggcccccaggaacccagaacttctctccagggaccccagcccgagcacccccttacccaggacccagccctgcccctcctcccctctgctctcctctcatcaccccatgggaatccggtatccccaggaagccatcaggaagggctgaaggaggaagcggggccgtgcaccaccgggcaggaggctccgtcttcgtgaacccagggaagtgccagcctcctagagggtatggtccaccctgcctggggctcccaccgtggcaggctgcggggaaggaccagggacggtgtgggggagggctcagggccctgcgggtgctcctccatcttcggtgagcctcccccttcacccaccgtcccgcccacctcctctccaccctggctgcacgtcttccacaccatcctgagtcctacctacaccagagccagcaaagccagtgcagacaaaggctggggtgcaggggggctgccagggcagcttcggggagggaaggatggagggaggggaggtcagtgaagaggcccccttcccctgggtccaggatcctcctctgggacccccggatcccatcccctcctggctctgggaggagaagcaggatgggagaatctgtgcgggaccctctcacagtggaatatccccacagcggctcaggccagacccaaaagcccctcagtgagccctccactgcagtcctgggcctgggtagcagcccctcccacagaggacagacccagcaccccgaagaagtcctgccagggggagctcagagccatgaaagagcaggatatggggtccccgatacaggcacagacctcagctccatccaggcccaccgggacccaccatgggaggaacacctgtctccgggttgtgaggtagctggcctctgtctcggaccccactccagacaccagacagaggggcaggccccccaaaaccagggttgagggatgatccgtcaaggcagacaagaccaaggggcactgaccccagcaagggaaggctcccaaacagacgaggaggattttgtagctgtctgtatcactgtgtgcaactgcagcagatgggctcgcgaccatagcaggtgctgccacagtgacactcgccaggtcaaaaaccccgtcccaagtcagcggaagcagagagagcagggaggacacgtttaggatctgaggccgcacctgacacccagggcagcagacgtctcccctccagggcaccctccaccgtcctgcgtttcttcaagaataggggcggcctgagggggtccagggccaggcgataggtcccctctaccccaaggaggagccaggcaggacccgagcaccgatgcatctaacgcagtcatgtaatgctgggtgacagtcagttcgcctacgta

SEQ ID NO: 235 - DNA, 12029 bp, synthetic construct
  misc_feature 1..12029: note = TxDH120126
  source 1..12029: mol_type = other DNA
tacgtaatgcatctaacgcagtcatgtaatgctgggtgacagtcagttcgcctccccattgaggctgacctgcccagacgggcctgggcccaccccacacaccggggcggaatgtgtgcaggccccagtctctgtgggtgttccgctagctggggcccccagtgctcaccccacacctaaagcgagccccagcctccagagccccctaagcattccccgcccagcagcccagcccctgcccccacccaggaggccccagagctcagggcgcctggtcggattttgtacagccccgagtcactgtggagagagcttgcaatggcagacgcggctgcagcagatgggctcgcgatcatagcaggtgctgccacagtgagaaaaactgtgtcaaaaaccgactcctggcagcagtcggaggccccgccagagaggggagcagccggcctgaacccatgtcctgccggttcccatgacccccagcacccagagccccacggtgtccccgttggataatgaggacaagggctgggggctccggtggtttgcggcagggacttgatcacatccttctgctgtggccccattgcctctggctggagttgacccttctgacaagtgtcctcagaaagacagggatcaccggcacctcccaatatcaaccccaggcagcacagacacaaaccccacatccagagccaactccaggagcagagacaccccaacactctgggggaccccaaccgtgataactccccactggaatccgccccagagtctaccaggaccaaaggccctgccctgtctctgtccctcactcagggcctcctgcagggcgagcgcttgggagcagactcggtcttaggggacaccactgtgggccccaactttgatgaggccactgacccttccttcctttcctggggcagcacagactttggggtctgggcagggaagaactactggctggtggccaatcacagagcccccaggccgaggtggccccaagaaggccctcaggaggtggccactccacttcctcccagctggaccccaggtcctccccaagataggggtgccatccaaggcaggtcctccatggagcccccttcagactcctcccgggaccccactggacctcagtccctgctctgggaatgcagccaccacaagcacaccaggaagcccaggcccagccaccctgcagtgggcaagcccacactctggagcagagcagggtgcgtctgggaggggctaacctccccaccccccaccccccatctgcacacagccacctaccactgcccagaccctctgcaggagggccaagccaccatggggtatggacttagggtctcactcacgtgcctcccctcctgggagaaggggcctcatgcccagatccctgcagcactagacacagctggaggcagtggccccagggccaccctgacctggcatctaaggctgctccagcccagacagcactgccgttcctgggaagcctgggctccaccagaccacaggtccagggcacagcccacaggagccacccacacacagctcacaggaagaagataagctccagaccccagggcgggacctgccttcctgccaccacttacacacaggccagggagctgttcccacacagatcaaccccaaaccgggactgcctggcactagggtcactgccatttccctctccattccctcccagtgcctctgtgctccctccttctggggaacaccctgtgcagcccctccctgcagcccacacgctggggagaccccaccctgcctcgggccttttctacctgctgcacttgccgcccacccaaacaaccctgggtacgtgaccctgcagtcctcaccctgatctgcaaccagacccctgtccctccctctaaacacccctcccaggccaactctgcacctgcaggccctccgctcttctgccacaagagcctcaggttttcctacctgtgcccaccccctaacccctcctgcccacaacttgagttcttcctctcctggagcccttgagccatggcactgaccctacactcccacccacacactgcccatgccatcaccttcctcctggacactctgaccccgctcccctccctctcagacccggccctggtatttccaggacaaaggctcacccaagtcttccccatgcaggcccttgccctcactgcctggttacacgggagcctcctgtgcgcagaagcagggagctcagctcttccacaggcagaaggcactgaaagaaatcagcctccagtgccttgacacacgtccgcctgtgtctctcactgcctgcacctgcagggaggctccgcactccctctaaagatgagggatccaggcagcaacatcacgggagaatgcagggctcccagacagcccagccctctcgcaggcctctcctgggaagagacctgcagccaccactgaacagccacggaggtcgctggatagtaaccgagtcagtgaccgacctggagggcaggggagcagtgaaccggagcccataccatagggacagagaccagccgctaacatcccgagcccctcactggcggccccagaacaccccgtggaaagagaacagacccacagtcccacctggaacagggcagacactgctgagcccccagcaccagccccaagaaacactaggcaacagcatcagagggggctcctgagaaagagaggaggggaggtctccttcaccatcaaatgcttcccttgaccaaaaacagggtccacgcaactcccccaggacaaaggaggagccccctgtacagcactgggctcagagtcctctctgagacaggctcagtttcagacaacaacccgctggaatgcacagtctcagcaggagagccaggccagagccagcaagaggagactcggtgacaccagtctcctgtagggacaggaggattttgtgggggttcgtgtcactgtgagcatattgtcggagcaggcagtgctattcccacagtgacacaaccccattcaaaaacccctactgcaaacgcacccactcctgggactgaggggctgggggagcgtctgggaagtatggcctaggggtgtccatcaatgcccaaaatgcaccagactctccccaagacatcaccccaccagccagtgagcagagtaaacagaaaatgagaagcagctgggaagcttgcacaggccccaaggaaagagctttggcaggtgtgcaagaggggatgtgggcagagcctcagcagggccttttgctgtttctgctttcctgtgcagagagttccataaactggtattcaagatcaatggctgggagtgagcccaggaggacagtgtgggaagagcacagggaaggaggagcagccgctatcctacactgtcatcttttgaaagtttgccctgtgcccacaatgctgcatcatgggatgcttaacagctgatgtagacacagctaaagagagaatcagtgaaatggatttgcagcacagatctgaataaatcctccagaatgtggagcagcacagaagcaagcacacagaaagtgcctgatgccaaggcaaagttcagtgggcaccttcaggcattgctgctgggcacagacactctgaaaagcactggcaggaactgcctgtgacaaagcagaaccctcaggcaatgccagccctagagcccttcctgagaacctcatgggcaaagatgtgcagaacagctgtttgtcatagccccaaactatggggctggacaaagcaaacgtccatctgaaggagaacagacaaataaacgatggcaggttcatgaaatgcaaactaggacagccagaggacaacagtagagagctacaggcggctttgcggttgagttcatgacaatgctgagtaattggagtaacagaggaaagcccaaaaaatacttttaatgtgatttcttctaaataaaatttacacccggcaaaatgaactatcttcttaagggataaactttcccctggaaaaactataaggaaaatcaagaaaacgatgatcacataaacacagtggtggttacttctactggggaaggaagagggtatgagctgagacacacagagtcggcaagtctcctaacaagaacagaacaaatacattacagtaccttgaaaacagcagttaaacttctaaatcgcaagaagaggaaaatgcacacacctgtgtttagaaaattctcagtccagcactgttcataatagcaaagacattaacccaggttggataaataagcgatgacacaggcaattgcacaatgatacagacatacattcagtatatgagacatcgatgatgtatccccaaagaaatgactttaaagagaaaaggcctgatgtgtggtggcaatcacctccctgggcatccccggacaggctgcaggctcactgtgtggcagggcaggcaggcacctgctggcagctcctggggcctgatgtggagcaggcacagagctgtatatccccaaggaaggtacagtcagtgcattccagagagaagcaactcagccacactccctggccagaacccaagatgcacacccatgcacagggaggcagagcccagcacctccgcagccaccaccacctgcgcacgggccaccaccttgcaggcacagagtgggtgctgagaggaggggcagggacaccaggcagggtgagcacccagagaaaactgcagaagcctcacacatccctcacctggcctgggcttcacctgacctggacctcacctggcctcgggcctcacctgcacctgctccaggtcttgctggagcctgagtagcactgaggctgtagggactcatccagggttggggaatgactctgcaactctcccacatctgacctttctgggtggaggcacctggtggcccagggaatataaaaagccccagaatgatgcctgtgtgatttgggggcaatttatgaacccgaaaggacatggccatggggtgggtagggacagtagggacagatgtcagcctgaggtgaagcctcaggacacaggtgggcatggacagtgtccacctaagcgagggacagacccgagtgtccctgcagtagacctgagagcgctgggcccacagcctcccctcggggccctgctgcctcctcaggtcagccctggacatcccgggtttccccaggcctggcggtaggattttgttgaggtctgtgtcactgtggtattactatgagaggcttgcttgtggcttccctaagagctgcagcaggcaagctaagcctcacagatgctgctattactaccacagtgtcacagagtccatcaaaaacccatgcctgggagcctcccaccacagccctccctgcgggggaccgctgcatgccgtgttaggattttgatcgaggacacggcgccatgggtatggtggctaccacagcagtgcagcccatgacccaaacacacggggcagcagaaacaatggacaggcccacaagtgaccatgatgggctccagcccaccagccccagagaccatgaaacagatggccaaggtcaccctacaggtcatccagatctggctccaaggggtctgcatcgctgctgccctcccaacgccaaaccagatggagacagggccggccccatagcaccatctgctgccgtccacccagcagtcccggaagcccctccctgaacgctgggccacgtgtgtgaaccctgcgagccccccatgtcagagtaggggcagcaggagggcggggctggccctgtgcactgtcactgcccctgtggtccctggcctgcctggccctgacacctgagcctctcctgggtcatttccaagacattcccagggacagccggagctgggagtcgctcatcctgcctggctgtcctgagtcctgctcatttccagacctcaccagggaagccaacagaggactcacctcacacagtcagagacaacgaaccttccagaaatccctgtttctctccccagtgagagaaaccctcttccagggtttctcttctctcccaccctcttccaggacagtcctcagcagcatcacagcgggaacgcacatctggatcaggacggcccccagaacacgcgatggcccatggggacagcccagcccttcccagacccctaaaaggtatccccaccttgcacctgccccagggctcaaactccaggaggcctgactcctgcacaccctcctgccagatatcacctcagccccctcctggaggggacaggagcccgggagggtgagtcagacccacctgccctcaatggcaggcggggaagattcagaaaggcctgagatccccaggacgcagcaccactgtcaatgggggccccagacgcctggaccagggcctgtgtgggaaaggcctctggccacactcagggggattttgtgaagggccctcccactgtggagaggctttgctgtggcttccctaagagctgccgcagcaggcaatgcaagcctcacagatgctgccacagtgatgaaaccagcatcaaaaaccgaccggactcgcagggtttatgcacacttctcggctcggagctctccaggagcacaagagccaggcccgagggtttgtgcccagaccctcggcctctagggacacccgggccatcttagccgatgggctgatgccctgcacaccgtgtgctgccaaacaggggcttcagagggctctgaggtgacttcactcatgaccacaggtgccctggtcccttcactgccagctgcaccagaccctgttccgagagatgccccagttccaaaagccaattcctggggccgggaattactgtagacaccagcctcattccagtacctcctgccaattgcctggattcccatcctggctggaatcaagagggcagcatccgccaggctcccaacaggcaggactcccacacaccctcctctgagaggccgctgtgttccgcagggccaggccgcagacagttcccctcacctgcccatgtagaaacacctgccattgtcgtccccacctggcaaagaccacttgtggagcccccagccccaggtacagctgtagagagagtcctcgaggcccctaagaaggagccatgcccagttctgccgggaccctcggccaggccgacaggagtggacgctggagctgggcccacactgggccacataggagctcaccagtgagggcaggagagcacatgccggggagcacccagcctcctgctgaccagagacccgtcccagagcccaggaggctgcagaggcctctccagggggacacagtgcatgtctggtccctgagcagcccccaggctctctagcactgggggcccctggcacagctgtctggaccctccctgttccctgggaagctcctcctgacagccccgcctccagttccaggtgtggattttgtcagggggtgccacactgtgtactgccagaagtggatgtggacttgcgatagtgagaggaagtgctgtgagggtatggtatgccggctgtggtgtaagaagaagctctggcacagtggtgccgcccatatcaaaaaccaggccaagtagacagacccctgccacgcagccccaggcctccagctcacctgcttctcctggggctctcaaggctgctgtctgccctctggccctctgtggggagggttccctcagtgggaggtctgtgctccagggcagggatgactgagatagaaatcaaaggctggcagggaaaggcagcttcccgccctgagaggtgcaggcagcaccacagagccatggagtcacagagccacggagcccccagtgtgggcgtgtgagggtgctgggctcccggcaggcccagccctgatggggaagcctgccccgtcccacagcccaggtccccaggggcagcaggcacagaagctgccaagctgtgctctacgatcctcatccctccagcagcatccactccacagtggggaaactgagccttggagaaccacccagccccctggaaacaaggcggggagcccagacagtgggcccagagcactgtgtgtatcctggcactaggtgcagggaccacccggagatccccatcactgagtggccagcctgcagaaggacccaaccccaaccaggccgcttgattaagctccatccccctgtcctgggaacctcttcccagcgccaccaacagctcggcttcccaggccctcatccctccaaggaaggccaaaggctgggcctgccaggggcacagtaccctcccttgccctggctaagacagggtgggcagacggctgcagataggacatattgctggggcatcttgctctgtgactactgggtactggctctcaacgcagaccctaccaaaatccccactgcctcccctgctaggggctggcctggtctcctcctgctgtcctaggaggctgctgacctccaggatggcttctgtccccagttctagggccagagcagatcccaggcaggctgtaggctgggaggccacccctgtccttgccgaggttcagtgcaggcacccaggacaggaaatggcctgaacacagggatgactgtgccatgccctacctaagtccgcccctttctactctgcaacccccactccccaggtcagcccatgacgaccaacaacccaacaccagagtcactgcctggccctgccctggggaggacccctcagcccccaccctgtctagaggagttggggggacaggacacaggctctctccttatggttcccccacctggctcctgccgggacccttggggtgtggacagaaaggacgcctgcctaattggcccccaggaacccagaacttctctccagggaccccagcccgagcacccccttacccaggacccagccctgcccctcctcccctctgctctcctctcatcactccatgggaatccagaatccccaggaagccatcaggaagggctgaaggaggaagcggggccgctgcaccaccgggcaggaggctccgtcttcgtgaacccagggaagtgccagcctcctagagggtatggtccaccctgcctggggctcccaccgtggcaggctgcggggaaggaccagggacggtgtgggggagggctcagggccctgcaggtgctccatcttggatgagcccatccctctcacccaccgacccgcccacctcctctccaccctggccacacgtcgtccacaccatcctgagtcccacctacaccagagccagcagagccagtgcagacagaggctggggtgcaggggggccgccagggcagctttggggagggaggaatggaggaaggggaggtcagtgaagaggcccccctcccctgggtctaggatccacctttgggacccccggatcccatcccctccaggctctgggaggagaagcaggatgggagattctgtgcaggaccctctcacagtggaatacctccacagcggctcaggccagatacaaaagcccctcagtgagccctccactgcagtgcagggcctgggggcagcccctcccacagaggacagacccagcaccccgaagaagtcctgccagggggagctcagagccatgaaggagcaagatatggggaccccaatactggcacagacctcagctccatccaggcccaccaggacccaccatgggtggaacacctgtctccggcccctgctggctgtgaggcagctggcctctgtctcggacccccattccagacaccagacagagggacaggccccccagaaccagtgttgagggacacccctgtccagggcagccaagtccaagaggcgcgctgagcccagcaagggaaggcccccaaacaaaccaggaggtttctgaagctgtctgtgtcacagtctgctgcaactgcagcagcaaatggtgccgcgaccatagcaggtgctgccacaatgacactgggcaggacagaaaccccatcccaagtcagccgaaggcagagagagcaggcaggacacatttaggatctgaggccacacctgacactcaagccaacagatgtctcccctccagggcgccctgccctgttcagtgttcctgagaaaacaggggcagcctgaggggatccagggccaggagatgggtcccctctaccccgaggaggagccaggcgggaatcccagccccctccccattgaggccatcctgcccagaggggcccggacccaccccacacacccaggcagaatgtgtgcaggcctcaggctctgtgggtgccgctagctggggctgccagtcctcaccccacacctaaggtgagccacagccgccagagcctccacaggagaccccacccagcagcccagcccctacccaggaggccccagagctcagggcgcctgggtggattttgtacagccccgagtcactgtgggtatagtggggagaggctttgtggcttccctaagagctgcagcaggcaaaagcctcacagatgctgcagctactaccacagtgagaaaagctatgtcaaaaaccgtctcccggccactgctggaggcccagccagagaagggaccagccgcccgaacatacgaccttcccagacctcatgacccccagcacttggagctccacagtgtccccattggatggtgaggatgggggccggggccatctgcacctcccaacatcacccccaggcagcacaggcacaaaccccaaatccagagccgacaccaggaacacagacaccccaataccctgggggaccctggccctggtgacttcccactgggatccacccccgtgtccacctggatcaaagaccccaccgctgtctctgtccctcactcagggcctgctgaggggcgggtgctttggagcagactcaggtttaggggccaccattgtggggcccaacctcgaccaggacacagatttttctttcctgccctggggcaacacagactttggggtctgtgcagggaggaccttctggaaagtcaccaagcacagagccctgactgaggtggtctcaggaagacccccaggagggggcttgtgccccttcctctcatgtggaccccatgccccccaagataggggcatcatgcagggcaggtcctccatgcagccaccactaggcaactccctggcgccggtccccactgcgcctccatcccggctctggggatgcagccaccatggccacaccaggcagcccgggtccagcaaccctgcagtgcccaagcccttggcaggattcccagaggctggagcccacccctcctcatccccccacacctgcacacacacacctaccccctgcccagtccccctccaggagggttggagccgcccatagggtgggggctccaggtctcactcactcgcttcccttcctgggcaaaggagcctcgtgccccggtcccccctgacggcgctgggcacaggtgtgggtactgggccccagggctcctccagccccagctgccctgctctccctgggaggcctgggcaccaccagaccaccagtccagggcacagccccagggagccgcccactgccagctcacaggaagaagataagcttcagaccctcagggccgggagctgccttcctgccaccccttcctgccccagacctccatgccctcccccaaccacttacacacaagccagggagctgtttccacacagttcaaccccaaaccaggacggcctggcactcgggtcactgccatttctgtctgcattcgctcccagcgcccctgtgttccctccctcctccctccttcctttcttcctgcattgggttcatgccgcagagtgccaggtgcaggtcagccctgagcttggggtcacctcctcactgaaggcagcctcagggtgcccaggggcaggcagggtgggggtgaggcttccagctccaaccgcttcgctaccttaggaccgttatagttaggcgcgccgtcgaccaattctcatgtttgacagcttatcatcgaatttctacgta

SEQ ID NO: 236 - DNA, 22 bp, synthetic construct
  misc_feature 1..22: note = Primer and/or probe
  source 1..22: mol_type = other DNA
tcttatcagacagggggctctc

SEQ ID NO: 237 - DNA, 55 bp, synthetic construct
  misc_feature 1..55: note = Primer and/or probe
  source 1..55: mol_type = other DNA
gtgactggagttcagacgtgtgctcttccgatcttcaccatggactgsacctgga

SEQ ID NO: 238 - DNA, 56 bp, synthetic construct
  misc_feature 1..56: note = Primer and/or probe
  source 1..56: mol_type = other DNA
gtgactggagttcagacgtgtgctcttccgatctccatggacacactttgytccac

SEQ ID NO: 239 - DNA, 57 bp, synthetic construct
  misc_feature 1..57: note = Primer and/or probe
  source 1..57: mol_type = other DNA
gtgactggagttcagacgtgtgctcttccgatcttcaccatggagtttgggctgagc

SEQ ID NO: 240 - DNA, 59 bp, synthetic construct
  misc_feature 1..59: note = Primer and/or probe
  source 1..59: mol_type = other DNA
gtgactggagttcagacgtgtgctcttccgatctagaacatgaaacayctgtggttctt

SEQ ID NO: 241 - DNA, 54 bp, synthetic construct
  misc_feature 1..54: note = Primer and/or probe
  source 1..54: mol_type = other DNA
gtgactggagttcagacgtgtgctcttccgatctatggggtcaaccgccatcct

SEQ ID NO: 242 - DNA, 57 bp, synthetic construct
  misc_feature 1..57: note = Primer and/or probe
  source 1..57: mol_type = other DNA
gtgactggagttcagacgtgtgctcttccgatctacaatgtctgtctccttcctcat

SEQ ID NO: 243 - DNA, 54 bp, synthetic construct
  misc_feature 1..54: note = Primer and/or probe
  source 1..54: mol_type = other DNA
acactctttccctacacgacgctcttccgatctgggaagacatttgggaaggac

SEQ ID NO: 244 - DNA, 64 bp, synthetic construct
  misc_feature 1..64: note = Primer and/or probe
  misc_feature 25..30: note = nnnnnn - 6 nucleotide index
  misc_feature 25..30: note = n is a, c, g, or t
  source 1..64: mol_type = other DNA
caagcagaagacggcatacgagatnnnnnngtgactggagttcagacgtgtgctcttccgatct

SEQ ID NO: 245 - DNA, 68 bp, synthetic construct
  misc_feature 1..68: note = Primer and/or probe
  misc_feature 29..35: note = nnnnnn - 6 nucleotide index
  misc_feature 30..35: note = n is a, c, g, or t
  source 1..68: mol_type = other DNA
aatgatacggcgaccaccgagatctacacnnnnnnacactctttccctacacgacgctcttccgatct